European Patent Specification EP 4 341 397 B1, published November 26, 2025. Title: Composition et methode permettant l'edition g nomique. Applicant: QUIDDITAS THERAPEUTICS. The sequence listing filed with the application follows.

SEQUENCE LISTING (646 sequences)

SEQ ID NO: 1 - DNA, 19 bp, Artificial sequence
  transposase binding site
ctgtctcttatacacatct

SEQ ID NO: 2 - DNA, 19 bp, Artificial sequence
  transposase binding site
agatgtgtataagagacag

SEQ ID NO: 3 - DNA, 19 bp, Artificial sequence
  transposase binding site
ctgactcttatacacaagt

SEQ ID NO: 4 - DNA, 19 bp, Artificial sequence
  transposase binding site
acttgtgtataagagtcag

SEQ ID NO: 5 - DNA, 19 bp, Artificial sequence
  transposase binding site
ctgtctcttgatcagatct

SEQ ID NO: 6 - DNA, 19 bp, Artificial sequence
  transposase binding site
agatctgatcaagagacag

SEQ ID NO: 7 - DNA, 167 bp, Artificial sequence
  premiere molecule de l'ensemble
  misc_feature (84)..(84): n is a, c, g, or t
tgcagctgctgtctcttatacacatcttttttttttttttttttttttttttttggcgatcgcttttttttttttttttttttnttttttttttttttttttttgcgatcgccttttttttttttttttgatacatgtttagatgtgtataagagacagctgtaagc

SEQ ID NO: 8 - DNA, 95 bp, Artificial sequence
  troisieme molecule de l'ensemble
  misc_feature (95)..(95): n= n'importe quel nucl otide ou un ou plusieurs sites de restriction
agatgtgtataagagacagcagctgcagacaaagcttacagctgtctcttatacacatctttttttttttttttttttttttcatatgccaagtn

SEQ ID NO: 9 - DNA, 189 bp, Artificial sequence
  deuxieme molecule de l'ensemble
  misc_feature (117)..(117): n is a, c, g, or t
atcatcctgtctcttatacacatcttttttttttttttttttgatagtagctgtctcttatacacatctttttttttttttttttttttttggcgatcgcttttttttttttttttnttttttttttttttttgcgatcgcctttttttttttttgatacatttagatgtgtataagagacaggatgat

SEQ ID NO: 10 - DNA, 64 bp, Artificial sequence
  troisieme molecule de l'ensemble
  misc_feature (1)..(1): n= n'importe quel nucl otide ou un ou plusieurs sites de restriction
nacttggttaattaattttttttttttttttttttttagatgtgtataagagacagctactatc

SEQ ID NO: 11 - DNA, 19 bp, Artificial sequence
  sequence de liaison Tn5
ctgtctcttatacacatct

SEQ ID NO: 12 - DNA, 33 bp, Artificial sequence
  sequence de liaison Tn5
tcgtcggcagcgtcagatgtgtataagagacag

SEQ ID NO: 13 - DNA, 34 bp, Artificial sequence
  sequence de liaison  Tn5
gtctcgtgggctcggagatgtgtataagagacag

SEQ ID NO: 14 - DNA, 22 bp, Artificial sequence
  oligo GFP sens
ctggtcgagctggacggcgacg

SEQ ID NO: 15 - DNA, 22 bp, Artificial sequence
  oligo GFP reverse
cacgaactccagcaggaccatg

SEQ ID NO: 16 - DNA, 21 bp, Artificial sequence
  oligo mCherry sens
aagggcgaggaggataacatg

SEQ ID NO: 17 - DNA, 18 bp, Artificial sequence
  oligo CD9 reverse
gaccatctcgcggttcct

SEQ ID NO: 18 - DNA, 32 bp, Artificial sequence
  oligo GFP Nde1 sens
acttggcatatgatggtgagcaagggcgagga

SEQ ID NO: 19 - DNA, 30 bp, Artificial sequence
  oligo GFP Nde1 reverse
acttggcatatgcttgtacagctcgtccat

SEQ ID NO: 20 - DNA, 32 bp, Artificial sequence
  oligo GFP BSPEI sens
tacaagtccggaatggtgagcaagggcgagga

SEQ ID NO: 21 - DNA, 30 bp, Artificial sequence
  oligo GFP BSPEI reverse
tacaagtccggacttgtacagctcgtccat

SEQ ID NO: 22 - DNA, 32 bp, Artificial sequence
  oligo CMV Nde1 sens
acttggcatatgccaagtacgccccctattga

SEQ ID NO: 23 - DNA, 86 bp, Artificial sequence
  oligo UVRD sens
ctcttcgctagctgccaccatgacgcgtggccccaagaaaaagcggaaagtgggaccggccaccatggacgtttcttacctgctcg

SEQ ID NO: 24 - DNA, 81 bp, Artificial sequence
  oligo UVRD reverse
aacaacacgtgccggtgatacccgcttccgcgcctgatccaccaccacctgacccaccaccagccaccgactccagccggg

SEQ ID NO: 25 - DNA, 29 bp, Artificial sequence
  oligo mSA sens
ctcttcgctagcgcggaagcgggtatcac

SEQ ID NO: 26 - DNA, 35 bp, Artificial sequence
  oligo mSA reverse
aacaagaattcttattatttaactttggtgaaggt

SEQ ID NO: 27 - DNA, 33 bp, Artificial sequence
  oligo Tn5 sens
ctcttcgctagcatgattaccagtgcactgcat

SEQ ID NO: 28 - DNA, 37 bp, Artificial sequence
  oligo Tn5 reverse
aacaagaattcttattagattttaatgccctgcgcca

SEQ ID NO: 29 - DNA, 6 bp, Artificial sequence
  restriction site
aacgtt

SEQ ID NO: 30 - DNA, 6 bp, Artificial sequence
  restriction site
aagctt

SEQ ID NO: 31 - DNA, 6 bp, Artificial sequence
  restriction site
aatatt

SEQ ID NO: 32 - DNA, 4 bp, Artificial sequence
  restriction site
aatt

SEQ ID NO: 33 - DNA, 6 bp, Artificial sequence
  restriction site
acatgt

SEQ ID NO: 34 - DNA, 6 bp, Artificial sequence
  restriction site
accggt

SEQ ID NO: 35 - DNA, 6 bp, Artificial sequence
  restriction site
acctgc

SEQ ID NO: 36 - DNA, 7 bp, Artificial sequence
  restriction site
accwggt

SEQ ID NO: 37 - DNA, 6 bp, Artificial sequence
  restriction site
acgcgt

SEQ ID NO: 38 - DNA, 5 bp, Artificial sequence
  restriction site
acggc

SEQ ID NO: 39 - DNA, 4 bp, Artificial sequence
  restriction site
acgt

SEQ ID NO: 40 - DNA, 5 bp, Artificial sequence
  restriction site
  misc_feature (3)..(3): n is a, c, g, or t
acngt

SEQ ID NO: 41 - DNA, 11 bp, Artificial sequence
  restriction site
  misc_feature (3)..(6): n is a, c, g, or t
acnnnngtayc

SEQ ID NO: 42 - DNA, 11 bp, Artificial sequence
  restriction site
  misc_feature (3)..(7): n is a, c, g, or t
acnnnnnctcc

SEQ ID NO: 43 - DNA, 6 bp, Artificial sequence
  restriction site
acrygt

SEQ ID NO: 44 - DNA, 6 bp, Artificial sequence
  restriction site
actagt

SEQ ID NO: 45 - DNA, 5 bp, Artificial sequence
  restriction site
actgg

SEQ ID NO: 46 - DNA, 6 bp, Artificial sequence
  restriction site
actggg

SEQ ID NO: 47 - DNA, 6 bp, Artificial sequence
  restriction site
agatct

SEQ ID NO: 48 - DNA, 6 bp, Artificial sequence
  restriction site
agcgct

SEQ ID NO: 49 - DNA, 4 bp, Artificial sequence
  restriction site
agct

SEQ ID NO: 50 - DNA, 6 bp, Artificial sequence
  restriction site
aggcct

SEQ ID NO: 51 - DNA, 6 bp, Artificial sequence
  restriction site
agtact

SEQ ID NO: 52 - DNA, 6 bp, Artificial sequence
  restriction site
atcgat

SEQ ID NO: 53 - DNA, 30 bp, Artificial sequence
  restriction site
atctatgtcgggtgcggagaaagaggtaat

SEQ ID NO: 54 - DNA, 6 bp, Artificial sequence
  restriction site
atgcat

SEQ ID NO: 55 - DNA, 6 bp, Artificial sequence
  restriction site
attaat

SEQ ID NO: 56 - DNA, 8 bp, Artificial sequence
  restriction site
atttaaat

SEQ ID NO: 57 - DNA, 12 bp, Artificial sequence
  restriction site
  misc_feature (4)..(8): n is a, c, g, or t
caannnnngtgg

SEQ ID NO: 58 - DNA, 6 bp, Artificial sequence
  restriction site
caattg

SEQ ID NO: 59 - DNA, 7 bp, Artificial sequence
  restriction site
cacctgc

SEQ ID NO: 60 - DNA, 6 bp, Artificial sequence
  restriction site
cacgag

SEQ ID NO: 61 - DNA, 6 bp, Artificial sequence
  restriction site
cacgag

SEQ ID NO: 62 - DNA, 6 bp, Artificial sequence
  restriction site
cacgtc

SEQ ID NO: 63 - DNA, 6 bp, Artificial sequence
  restriction site
cacgtg

SEQ ID NO: 64 - DNA, 9 bp, Artificial sequence
  restriction site
  misc_feature (4)..(6): n is a, c, g, or t
cacnnngtg

SEQ ID NO: 65 - DNA, 10 bp, Artificial sequence
  restriction site
  misc_feature (4)..(7): n is a, c, g, or t
cacnnnngtg

SEQ ID NO: 66 - DNA, 6 bp, Artificial sequence
  restriction site
cagcag

SEQ ID NO: 67 - DNA, 6 bp, Artificial sequence
  restriction site
cagctg

SEQ ID NO: 68 - DNA, 9 bp, Artificial sequence
  restriction site
  misc_feature (4)..(6): n is a, c, g, or t
cagnnnctg

SEQ ID NO: 69 - DNA, 5 bp, Artificial sequence
  restriction site
cagtg

SEQ ID NO: 70 - DNA, 6 bp, Artificial sequence
  restriction site
catatg

SEQ ID NO: 71 - DNA, 4 bp, Artificial sequence
  restriction site
catg

SEQ ID NO: 72 - DNA, 4 bp, Artificial sequence
  restriction site
catg

SEQ ID NO: 73 - DNA, 4 bp, Artificial sequence
  restriction site
catg

SEQ ID NO: 74 - DNA, 10 bp, Artificial sequence
  restriction site
  misc_feature (4)..(7): n is a, c, g, or t
caynnnnrtg

SEQ ID NO: 75 - DNA, 15 bp, Artificial sequence
  restriction site
  misc_feature (4)..(12): n is a, c, g, or t
ccannnnnnnnntgg

SEQ ID NO: 76 - DNA, 12 bp, Artificial sequence
  restriction site
  misc_feature (4)..(9): n is a, c, g, or t
ccannnnnntgg

SEQ ID NO: 77 - DNA, 11 bp, Artificial sequence
  restriction site
  misc_feature (4)..(8): n is a, c, g, or t
ccannnnntgg

SEQ ID NO: 78 - DNA, 5 bp, Artificial sequence
  restriction site
ccatc

SEQ ID NO: 79 - DNA, 6 bp, Artificial sequence
  restriction site
ccatgg

SEQ ID NO: 80 - DNA, 6 bp, Artificial sequence
  restriction site
cccagc

SEQ ID NO: 81 - DNA, 5 bp, Artificial sequence
  restriction site
cccgc

SEQ ID NO: 82 - DNA, 6 bp, Artificial sequence
  restriction site
cccggg

SEQ ID NO: 83 - DNA, 6 bp, Artificial sequence
  restriction site
cccggg

SEQ ID NO: 84 - DNA, 4 bp, Artificial sequence
  restriction site
ccdg

SEQ ID NO: 85 - DNA, 4 bp, Artificial sequence
  restriction site
ccgc

SEQ ID NO: 86 - DNA, 6 bp, Artificial sequence
  restriction site
ccgcgg

SEQ ID NO: 87 - DNA, 6 bp, Artificial sequence
  restriction site
ccgctc

SEQ ID NO: 88 - DNA, 4 bp, Artificial sequence
  restriction site
ccgg

SEQ ID NO: 89 - DNA, 5 bp, Artificial sequence
  restriction site
  misc_feature (3)..(3): n is a, c, g, or t
ccngg

SEQ ID NO: 90 - DNA, 5 bp, Artificial sequence
  restriction site
  misc_feature (3)..(3): n is a, c, g, or t
ccngg

SEQ ID NO: 91 - DNA, 6 bp, Artificial sequence
  restriction site
  misc_feature (3)..(4): n is a, c, g, or t
ccnngg

SEQ ID NO: 92 - DNA, 11 bp, Artificial sequence
  restriction site
  misc_feature (3)..(9): n is a, c, g, or t
ccnnnnnnngg

SEQ ID NO: 93 - DNA, 6 bp, Artificial sequence
  restriction site
ccrygg

SEQ ID NO: 94 - DNA, 5 bp, Artificial sequence
  restriction site
ccsgg

SEQ ID NO: 95 - DNA, 6 bp, Artificial sequence
  restriction site
cctagg

SEQ ID NO: 96 - DNA, 4 bp, Artificial sequence
  restriction site
cctc

SEQ ID NO: 97 - DNA, 7 bp, Artificial sequence
  restriction site
cctcagc

SEQ ID NO: 98 - DNA, 7 bp, Artificial sequence
  restriction site
cctcagc

SEQ ID NO: 99 - DNA, 7 bp, Artificial sequence
  restriction site
cctcagc

SEQ ID NO: 100 - DNA, 8 bp, Artificial sequence
  restriction site
cctgcagg

SEQ ID NO: 101 - DNA, 7 bp, Artificial sequence
  restriction site
  misc_feature (4)..(4): n is a, c, g, or t
cctnagc

SEQ ID NO: 102 - DNA, 7 bp, Artificial sequence
  restriction site
  misc_feature (4)..(4): n is a, c, g, or t
cctnagg

SEQ ID NO: 103 - DNA, 11 bp, Artificial sequence
  restriction site
  misc_feature (4)..(8): n is a, c, g, or t
cctnnnnnagg

SEQ ID NO: 104 - DNA, 5 bp, Artificial sequence
  restriction site
ccttc

SEQ ID NO: 105 - DNA, 5 bp, Artificial sequence
  restriction site
ccwgg

SEQ ID NO: 106 - DNA, 5 bp, Artificial sequence
  restriction site
ccwgg

SEQ ID NO: 107 - DNA, 6 bp, Artificial sequence
  restriction site
ccwwgg

SEQ ID NO: 108 - DNA, 12 bp, Artificial sequence
  restriction site
  misc_feature (4)..(9): n is a, c, g, or t
cgannnnnntgc

SEQ ID NO: 109 - DNA, 6 bp, Artificial sequence
  restriction site
cgatcg

SEQ ID NO: 110 - DNA, 4 bp, Artificial sequence
  restriction site
cgcg

SEQ ID NO: 111 - DNA, 6 bp, Artificial sequence
  restriction site
cggccg

SEQ ID NO: 112 - DNA, 7 bp, Artificial sequence
  restriction site
cggwccg

SEQ ID NO: 113 - DNA, 6 bp, Artificial sequence
  restriction site
cgrycg

SEQ ID NO: 114 - DNA, 6 bp, Artificial sequence
  restriction site
cgtacg

SEQ ID NO: 115 - DNA, 6 bp, Artificial sequence
  restriction site
cgtctc

SEQ ID NO: 116 - DNA, 6 bp, Artificial sequence
  restriction site
cgtctc

SEQ ID NO: 117 - DNA, 5 bp, Artificial sequence
  restriction site
cgwcg

SEQ ID NO: 118 - DNA, 6 bp, Artificial sequence
  restriction site
cmgckg

SEQ ID NO: 119 - DNA, 22 bp, Artificial sequence
  restriction site
  misc_feature (2)..(21): n is a, c, g, or t
cnnnnnnnnnnnnnnnnnnnng

SEQ ID NO: 120 - DNA, 4 bp, Artificial sequence
  restriction site
  misc_feature (2)..(3): n is a, c, g, or t
cnnr

SEQ ID NO: 121 - DNA, 8 bp, Artificial sequence
  restriction site
crccggyg

SEQ ID NO: 122 - DNA, 4 bp, Artificial sequence
  restriction site
ctag

SEQ ID NO: 123 - DNA, 5 bp, Artificial sequence
  restriction site
ctcag

SEQ ID NO: 124 - DNA, 6 bp, Artificial sequence
  restriction site
ctcgag

SEQ ID NO: 125 - DNA, 6 bp, Artificial sequence
  restriction site
ctcttc

SEQ ID NO: 126 - DNA, 6 bp, Artificial sequence
  restriction site
ctgaag

SEQ ID NO: 127 - DNA, 6 bp, Artificial sequence
  restriction site
ctgcag

SEQ ID NO: 128 - DNA, 6 bp, Artificial sequence
  restriction site
ctggag

SEQ ID NO: 129 - DNA, 5 bp, Artificial sequence
  restriction site
  misc_feature (3)..(3): n is a, c, g, or t
ctnag

SEQ ID NO: 130 - DNA, 6 bp, Artificial sequence
  restriction site
ctryag

SEQ ID NO: 131 - DNA, 6 bp, Artificial sequence
  restriction site
cttaag

SEQ ID NO: 132 - DNA, 6 bp, Artificial sequence
  restriction site
cttgag

SEQ ID NO: 133 - DNA, 6 bp, Artificial sequence
  restriction site
ctyrag

SEQ ID NO: 134 - DNA, 6 bp, Artificial sequence
  restriction site
cycgrg

SEQ ID NO: 135 - DNA, 5 bp, Artificial sequence
  restriction site
gaaga

SEQ ID NO: 136 - DNA, 6 bp, Artificial sequence
  restriction site
gaagac

SEQ ID NO: 137 - DNA, 10 bp, Artificial sequence
  restriction site
  misc_feature (4)..(7): n is a, c, g, or t
gaannnnttc

SEQ ID NO: 138 - DNA, 6 bp, Artificial sequence
  restriction site
gaatgc

SEQ ID NO: 139 - DNA, 6 bp, Artificial sequence
  restriction site
gaatgc

SEQ ID NO: 140 - DNA, 6 bp, Artificial sequence
  restriction site
gaattc

SEQ ID NO: 141 - DNA, 5 bp, Artificial sequence
  restriction site
gacgc

SEQ ID NO: 142 - DNA, 6 bp, Artificial sequence
  restriction site
gacgtc

SEQ ID NO: 143 - DNA, 6 bp, Artificial sequence
  restriction site
gacgtc

SEQ ID NO: 144 - DNA, 9 bp, Artificial sequence
  restriction site
  misc_feature (4)..(6): n is a, c, g, or t
gacnnngtc

SEQ ID NO: 145 - DNA, 10 bp, Artificial sequence
  restriction site
  misc_feature (4)..(7): n is a, c, g, or t
gacnnnngtc

SEQ ID NO: 146 - DNA, 11 bp, Artificial sequence
  restriction site
  misc_feature (4)..(8): n is a, c, g, or t
gacnnnnngtc

SEQ ID NO: 147 - DNA, 12 bp, Artificial sequence
  restriction site
  misc_feature (4)..(9): n is a, c, g, or t
gacnnnnnngtc

SEQ ID NO: 148 - DNA, 6 bp, Artificial sequence
  restriction site
gagctc

SEQ ID NO: 149 - DNA, 6 bp, Artificial sequence
  restriction site
gagctc

SEQ ID NO: 150 - DNA, 6 bp, Artificial sequence
  restriction site
gaggag

SEQ ID NO: 151 - DNA, 5 bp, Artificial sequence
  restriction site
gagtc

SEQ ID NO: 152 - DNA, 5 bp, Artificial sequence
  restriction site
gagtc

SEQ ID NO: 153 - DNA, 5 bp, Artificial sequence
  restriction site
gagtc

SEQ ID NO: 154 - DNA, 5 bp, Artificial sequence
  restriction site
  misc_feature (3)..(3): n is a, c, g, or t
gantc

SEQ ID NO: 155 - DNA, 6 bp, Artificial sequence
  restriction site
gatatc

SEQ ID NO: 156 - DNA, 4 bp, Artificial sequence
  restriction site
gatc

SEQ ID NO: 157 - DNA, 4 bp, Artificial sequence
  restriction site
gatc

SEQ ID NO: 158 - DNA, 10 bp, Artificial sequence
  restriction site
  misc_feature (4)..(7): n is a, c, g, or t
gatnnnnatc

SEQ ID NO: 159 - DNA, 5 bp, Artificial sequence
  restriction site
gawtc

SEQ ID NO: 160 - DNA, 6 bp, Artificial sequence
  restriction site
gcaatg

SEQ ID NO: 161 - DNA, 6 bp, Artificial sequence
  restriction site
gcaatg

SEQ ID NO: 162 - DNA, 5 bp, Artificial sequence
  restriction site
gcagc

SEQ ID NO: 163 - DNA, 6 bp, Artificial sequence
  restriction site
gcagtg

SEQ ID NO: 164 - DNA, 6 bp, Artificial sequence
  restriction site
gcagtg

SEQ ID NO: 165 - DNA, 11 bp, Artificial sequence
  restriction site
  misc_feature (4)..(8): n is a, c, g, or t
gcannnnntgc

SEQ ID NO: 166 - DNA, 5 bp, Artificial sequence
  restriction site
gcatc

SEQ ID NO: 167 - DNA, 6 bp, Artificial sequence
  restriction site
gcatgc

SEQ ID NO: 168 - DNA, 8 bp, Artificial sequence
  restriction site
gcccgggc

SEQ ID NO: 169 - DNA, 6 bp, Artificial sequence
  restriction site
gccgag

SEQ ID NO: 170 - DNA, 6 bp, Artificial sequence
  restriction site
gccggc

SEQ ID NO: 171 - DNA, 6 bp, Artificial sequence
  restriction site
gccggc

SEQ ID NO: 172 - DNA, 11 bp, Artificial sequence
  restriction site
  misc_feature (4)..(8): n is a, c, g, or t
gccnnnnnggc

SEQ ID NO: 173 - DNA, 8 bp, Artificial sequence
  restriction site
gcgatcgc

SEQ ID NO: 174 - DNA, 6 bp, Artificial sequence
  restriction site
gcgatg

SEQ ID NO: 175 - DNA, 4 bp, Artificial sequence
  restriction site
gcgc

SEQ ID NO: 176 - DNA, 4 bp, Artificial sequence
  restriction site
gcgc

SEQ ID NO: 177 - DNA, 6 bp, Artificial sequence
  restriction site
gcgcgc

SEQ ID NO: 178 - DNA, 8 bp, Artificial sequence
  restriction site
gcggccgc

SEQ ID NO: 179 - DNA, 5 bp, Artificial sequence
  restriction site
  misc_feature (3)..(3): n is a, c, g, or t
gcngc

SEQ ID NO: 180 - DNA, 6 bp, Artificial sequence
  restriction site
  misc_feature (3)..(4): n is a, c, g, or t
gcnngc

SEQ ID NO: 181 - DNA, 11 bp, Artificial sequence
  restriction site
  misc_feature (3)..(9): n is a, c, g, or t
gcnnnnnnngc

SEQ ID NO: 182 - DNA, 6 bp, Artificial sequence
  restriction site
gctagc

SEQ ID NO: 183 - DNA, 6 bp, Artificial sequence
  restriction site
gctagc

SEQ ID NO: 184 - DNA, 7 bp, Artificial sequence
  restriction site
gctcttc

SEQ ID NO: 185 - DNA, 7 bp, Artificial sequence
  restriction site
gctcttc

SEQ ID NO: 186 - DNA, 7 bp, Artificial sequence
  restriction site
  misc_feature (4)..(4): n is a, c, g, or t
gctnagc

SEQ ID NO: 187 - DNA, 5 bp, Artificial sequence
  restriction site
gcwgc

SEQ ID NO: 188 - DNA, 6 bp, Artificial sequence
  restriction site
gdgchc

SEQ ID NO: 189 - DNA, 5 bp, Artificial sequence
  restriction site
ggatc

SEQ ID NO: 190 - DNA, 5 bp, Artificial sequence
  restriction site
ggatc

SEQ ID NO: 191 - DNA, 6 bp, Artificial sequence
  restriction site
ggatcc

SEQ ID NO: 192 - DNA, 5 bp, Artificial sequence
  restriction site
ggatg

SEQ ID NO: 193 - DNA, 5 bp, Artificial sequence
  restriction site
ggatg

SEQ ID NO: 194 - DNA, 4 bp, Artificial sequence
  restriction site
ggcc

SEQ ID NO: 195 - DNA, 8 bp, Artificial sequence
  restriction site
ggccggcc

SEQ ID NO: 196 - DNA, 13 bp, Artificial sequence
  restriction site
  misc_feature (5)..(9): n is a, c, g, or t
ggccnnnnnggcc

SEQ ID NO: 197 - DNA, 6 bp, Artificial sequence
  restriction site
ggcgcc

SEQ ID NO: 198 - DNA, 6 bp, Artificial sequence
  restriction site
ggcgcc

SEQ ID NO: 199 - DNA, 6 bp, Artificial sequence
  restriction site
ggcgcc

SEQ ID NO: 200 - DNA, 6 bp, Artificial sequence
  restriction site
ggcgcc

SEQ ID NO: 201 - DNA, 8 bp, Artificial sequence
  restriction site
ggcgcgcc

SEQ ID NO: 202 - DNA, 6 bp, Artificial sequence
  restriction site
ggcgga

SEQ ID NO: 203 - DNA, 5 bp, Artificial sequence
  restriction site
gggac

SEQ ID NO: 204 - DNA, 6 bp, Artificial sequence
  restriction site
gggccc

SEQ ID NO: 205 - DNA, 6 bp, Artificial sequence
  restriction site
gggccc

SEQ ID NO: 206 - DNA, 5 bp, Artificial sequence
  restriction site
  misc_feature (3)..(3): n is a, c, g, or t
ggncc

SEQ ID NO: 207 - DNA, 6 bp, Artificial sequence
  restriction site
  misc_feature (3)..(4): n is a, c, g, or t
ggnncc

SEQ ID NO: 208 - DNA, 6 bp, Artificial sequence
  restriction site
ggtacc

SEQ ID NO: 209 - DNA, 6 bp, Artificial sequence
  restriction site
ggtacc

SEQ ID NO: 210 - DNA, 6 bp, Artificial sequence
  restriction site
ggtctc

SEQ ID NO: 211 - DNA, 5 bp, Artificial sequence
  restriction site
ggtga

SEQ ID NO: 212 - DNA, 7 bp, Artificial sequence
  restriction site
  misc_feature (4)..(4): n is a, c, g, or t
ggtnacc

SEQ ID NO: 213 - DNA, 5 bp, Artificial sequence
  restriction site
ggwcc

SEQ ID NO: 214 - DNA, 6 bp, Artificial sequence
  restriction site
ggyrcc

SEQ ID NO: 215 - DNA, 6 bp, Artificial sequence
  restriction site
gkgcmc

SEQ ID NO: 216 - DNA, 6 bp, Artificial sequence
  restriction site
grcgyc

SEQ ID NO: 217 - DNA, 6 bp, Artificial sequence
  restriction site
grgcyc

SEQ ID NO: 218 - DNA, 4 bp, Artificial sequence
  restriction site
gtac

SEQ ID NO: 219 - DNA, 4 bp, Artificial sequence
  restriction site
gtac

SEQ ID NO: 220 - DNA, 6 bp, Artificial sequence
  restriction site
gtatac

SEQ ID NO: 221 - DNA, 6 bp, Artificial sequence
  restriction site
gtatcc

SEQ ID NO: 222 - DNA, 6 bp, Artificial sequence
  restriction site
gtcgac

SEQ ID NO: 223 - DNA, 5 bp, Artificial sequence
  restriction site
gtctc

SEQ ID NO: 224 - DNA, 5 bp, Artificial sequence
  restriction site
gtctc

SEQ ID NO: 225 - DNA, 6 bp, Artificial sequence
  restriction site
gtgcac

SEQ ID NO: 226 - DNA, 6 bp, Artificial sequence
  restriction site
gtgcag

SEQ ID NO: 227 - DNA, 6 bp, Artificial sequence
  restriction site
gtmkac

SEQ ID NO: 228 - DNA, 6 bp, Artificial sequence
  restriction site
  misc_feature (3)..(4): n is a, c, g, or t
gtnnac

SEQ ID NO: 229 - DNA, 5 bp, Artificial sequence
  restriction site
gtsac

SEQ ID NO: 230 - DNA, 6 bp, Artificial sequence
  restriction site
gttaac

SEQ ID NO: 231 - DNA, 8 bp, Artificial sequence
  restriction site
gtttaaac

SEQ ID NO: 232 - DNA, 6 bp, Artificial sequence
  restriction site
gtyrac

SEQ ID NO: 233 - DNA, 6 bp, Artificial sequence
  restriction site
gwgcwc

SEQ ID NO: 234 - DNA, 9 bp, Artificial sequence
  restriction site
  misc_feature (1)..(2): n is a, c, g, or t
  misc_feature (8)..(9): n is a, c, g, or t
nncastgnn

SEQ ID NO: 235 - DNA, 6 bp, Artificial sequence
  restriction site
raatty

SEQ ID NO: 236 - DNA, 6 bp, Artificial sequence
  restriction site
rcatgy

SEQ ID NO: 237 - DNA, 6 bp, Artificial sequence
  restriction site
rccggy

SEQ ID NO: 238 - DNA, 6 bp, Artificial sequence
  restriction site
rgatcy

SEQ ID NO: 239 - DNA, 6 bp, Artificial sequence
  restriction site
rgcgcy

SEQ ID NO: 240 - DNA, 4 bp, Artificial sequence
  restriction site
rgcy

SEQ ID NO: 241 - DNA, 7 bp, Artificial sequence
  restriction site
  misc_feature (4)..(4): n is a, c, g, or t
rggnccy

SEQ ID NO: 242 - DNA, 7 bp, Artificial sequence
  restriction site
rggwccy

SEQ ID NO: 243 - DNA, 27 bp, Artificial sequence
  restriction site
taactataacggtcctaaggtagcgaa

SEQ ID NO: 244 - DNA, 6 bp, Artificial sequence
  restriction site
tacgta

SEQ ID NO: 245 - DNA, 18 bp, Artificial sequence
  restriction site
tagggataacagggtaat

SEQ ID NO: 246 - DNA, 6 bp, Artificial sequence
  restriction site
tcatga

SEQ ID NO: 247 - DNA, 6 bp, Artificial sequence
  restriction site
tccgga

SEQ ID NO: 248 - DNA, 6 bp, Artificial sequence
  restriction site
tccrac

SEQ ID NO: 249 - DNA, 4 bp, Artificial sequence
  restriction site
tcga

SEQ ID NO: 250 - DNA, 6 bp, Artificial sequence
  restriction site
tcgcga

SEQ ID NO: 251 - DNA, 5 bp, Artificial sequence
  restriction site
  misc_feature (3)..(3): n is a, c, g, or t
tcnga

SEQ ID NO: 252 - DNA, 6 bp, Artificial sequence
  restriction site
  misc_feature (3)..(4): n is a, c, g, or t
tcnnga

SEQ ID NO: 253 - DNA, 6 bp, Artificial sequence
  restriction site
tctaga

SEQ ID NO: 254 - DNA, 6 bp, Artificial sequence
  restriction site
tgatca

SEQ ID NO: 255 - DNA, 4 bp, Artificial sequence
  restriction site
tgca

SEQ ID NO: 256 - DNA, 6 bp, Artificial sequence
  restriction site
tgcgca

SEQ ID NO: 257 - DNA, 30 bp, Artificial sequence
  restriction site
tggcaaacagctattatgggtattatgggt

SEQ ID NO: 258 - DNA, 6 bp, Artificial sequence
  restriction site
tggcca

SEQ ID NO: 259 - DNA, 6 bp, Artificial sequence
  restriction site
tgtaca

SEQ ID NO: 260 - DNA, 4 bp, Artificial sequence
  restriction site
ttaa

SEQ ID NO: 261 - DNA, 8 bp, Artificial sequence
  restriction site
ttaattaa

SEQ ID NO: 262 - DNA, 6 bp, Artificial sequence
  restriction site
ttataa

SEQ ID NO: 263 - DNA, 6 bp, Artificial sequence
  restriction site
ttcgaa

SEQ ID NO: 264 - DNA, 6 bp, Artificial sequence
  restriction site
tttaaa

SEQ ID NO: 265 - DNA, 8 bp, Artificial sequence
  restriction site
vctcgagb

SEQ ID NO: 266 - DNA, 6 bp, Artificial sequence
  restriction site
wccggw

SEQ ID NO: 267 - DNA, 6 bp, Artificial sequence
  restriction site
yacgtr

SEQ ID NO: 268 - DNA, 6 bp, Artificial sequence
  restriction site
yggccr

SEQ ID NO: 269 - DNA, 20 bp, Artificial sequence
  transposase binding site
ctgagagatcccctcataat

SEQ ID NO: 270 - DNA, 20 bp, Artificial sequence
  transposase binding site
attatgaggggatctctcag

SEQ ID NO: 271 - DNA, 20 bp, Artificial sequence
  transposase binding site
gactctctaggggagtatta

SEQ ID NO: 272 - DNA, 20 bp, Artificial sequence
  transposase binding site
taatactcccctagagagtc

SEQ ID NO: 273 - DNA, 20 bp, Artificial sequence
  transposase binding site
ctgagagatcccctcataat

SEQ ID NO: 274 - DNA, 20 bp, Artificial sequence
  transposase binding site
attatgaggggatctctcag

SEQ ID NO: 275 - DNA, 20 bp, Artificial sequence
  transposase binding site
gactctctaggggagtatta

SEQ ID NO: 276 - DNA, 20 bp, Artificial sequence
  transposase binding site
taatactcccctagagagtc

SEQ ID NO: 277 - DNA, 20 bp, Artificial sequence
  transposase binding site
ctgagagatcccctcataat

SEQ ID NO: 278 - DNA, 20 bp, Artificial sequence
  transposase binding site
attatgaggggatctctcag

SEQ ID NO: 279 - DNA, 20 bp, Artificial sequence
  transposase binding site
gactctctaggggagtatta

SEQ ID NO: 280 - DNA, 20 bp, Artificial sequence
  transposase binding site
taatactcccctagagagtc

SEQ ID NO: 281 - DNA, 20 bp, Artificial sequence
  transposase binding site
ctgagagatcccctcataat

SEQ ID NO: 282 - DNA, 20 bp, Artificial sequence
  transposase binding site
attatgaggggatctctcag

SEQ ID NO: 283 - DNA, 20 bp, Artificial sequence
  transposase binding site
gactctctaggggagtatta

SEQ ID NO: 284 - DNA, 20 bp, Artificial sequence
  transposase binding site
taatactcccctagagagtc

SEQ ID NO: 285 - DNA, 29 bp, Artificial sequence
  transposase binding site
ctgatgaatcccctaatgattttggtaaa

SEQ ID NO: 286 - DNA, 29 bp, Artificial sequence
  transposase binding site
tttaccaaaatcattaggggattcatcag

SEQ ID NO: 287 - DNA, 29 bp, Artificial sequence
  transposase binding site
ctgagagatcccctcataatttccccaaa

SEQ ID NO: 288 - DNA, 29 bp, Artificial sequence
  transposase binding site
tttggggaaattatgaggggatctctcag

SEQ ID NO: 289 - DNA, 29 bp, Artificial sequence
  transposase binding site
catggccgtcaacctaagaagccttattt

SEQ ID NO: 290 - DNA, 29 bp, Artificial sequence
  transposase binding site
aaataaggcttcttaggttgacggccatg

SEQ ID NO: 291 - DNA, 29 bp, Artificial sequence
  transposase binding site
catggccgtcaacctaagaaggcataaaa

SEQ ID NO: 292 - DNA, 29 bp, Artificial sequence
  transposase binding site
ttttatgccttcttaggttgacggccatg

SEQ ID NO: 293 - DNA, 29 bp, Artificial sequence
  transposase binding site
cactacagttgcattttgtgttgagttct

SEQ ID NO: 294 - DNA, 29 bp, Artificial sequence
  transposase binding site
agaactcaacacaaaatgcaactgtagtg

SEQ ID NO: 295 - DNA, 29 bp, Artificial sequence
  transposase binding site
cactacagttgcattttgtgtcgtgagtg

SEQ ID NO: 296 - DNA, 29 bp, Artificial sequence
  transposase binding site
cactcacgacacaaaatgcaactgtagtg

SEQ ID NO: 297 - DNA, 29 bp, Artificial sequence
  transposase binding site
cataagcgctaacttaagggttgtggtat

SEQ ID NO: 298 - DNA, 29 bp, Artificial sequence
  transposase binding site
ataccacaacccttaagttagcgcttatg

SEQ ID NO: 299 - DNA, 29 bp, Artificial sequence
  transposase binding site
cataagcgctaacttaagggttgaaccat

SEQ ID NO: 300 - DNA, 29 bp, Artificial sequence
  transposase binding site
atggttcaacccttaagttagcgcttatg

SEQ ID NO: 301 - DNA, 29 bp, Artificial sequence
  transposase binding site
catgcccatcaacttaagaatctagacta

SEQ ID NO: 302 - DNA, 29 bp, Artificial sequence
  transposase binding site
tagtctagattcttaagttgatgggcatg

SEQ ID NO: 303 - DNA, 29 bp, Artificial sequence
  transposase binding site
catgcccatcaacttaagaacaaaaataa

SEQ ID NO: 304 - DNA, 29 bp, Artificial sequence
  transposase binding site
ttatttttgttcttaagttgatgggcatg

SEQ ID NO: 305 - DNA, 29 bp, Artificial sequence
  transposase binding site
catcgccatcaagctaaggaaaaggagat

SEQ ID NO: 306 - DNA, 29 bp, Artificial sequence
  transposase binding site
atctccttttccttagcttgatggcgatg

SEQ ID NO: 307 - DNA, 29 bp, Artificial sequence
  transposase binding site
catcgccatcaagctaacgaaattgaact

SEQ ID NO: 308 - DNA, 29 bp, Artificial sequence
  transposase binding site
agttcaatttcgttagcttgatggcgatg

SEQ ID NO: 309 - DNA, 29 bp, Artificial sequence
  transposase binding site
taatgccgatcagttaaggatcagttcac

SEQ ID NO: 310 - DNA, 29 bp, Artificial sequence
  transposase binding site
gtgaactgatccttaactgatcggcatta

SEQ ID NO: 311 - DNA, 29 bp, Artificial sequence
  transposase binding site
taatgccagtcagttaagcaactgactgg

SEQ ID NO: 312 - DNA, 29 bp, Artificial sequence
  transposase binding site
ccagtcagttgcttaactgactggcatta

SEQ ID NO: 313 - DNA, 29 bp, Artificial sequence
  transposase binding site
taagagagttaatttataatctattttca

SEQ ID NO: 314 - DNA, 29 bp, Artificial sequence
  transposase binding site
tgaaaatagattataaattaactctctta

SEQ ID NO: 315 - DNA, 29 bp, Artificial sequence
  transposase binding site
taaggatgttaatttattaatttaaaagg

SEQ ID NO: 316 - DNA, 29 bp, Artificial sequence
  transposase binding site
ccttttaaattaataaattaacatcctta

SEQ ID NO: 317 - DNA, 29 bp, Artificial sequence
  transposase binding site
ctgactcttatacacaagtagcgtcctga

SEQ ID NO: 318 - DNA, 29 bp, Artificial sequence
  transposase binding site
tcaggacgctacttgtgtataagagtcag

SEQ ID NO: 319 - DNA, 30 bp, Artificial sequence
  transposase binding site
caggcgtgttgattatccaataaaatccca

SEQ ID NO: 320 - DNA, 29 bp, Artificial sequence
  transposase binding site
caggggatcaagatctgatcaagagacag

SEQ ID NO: 321 - DNA, 30 bp, Artificial sequence; identical to SEQ ID NO: 319
  transposase binding site

SEQ ID NO: 322 - DNA, 30 bp, Artificial sequence
  transposase binding site
tgggattttattggataatcaacacgcctg

SEQ ID NO: 323 - DNA, 30 bp, Artificial sequence
  transposase binding site
cacgagtgttgattatccaaaattataaca

SEQ ID NO: 324 - DNA, 30 bp, Artificial sequence
  transposase binding site
tgttataattttggataatcaacactcgtg

SEQ ID NO: 325 - DNA, 30 bp, Artificial sequence
  transposase binding site
cttaacgggtgacaaggcatcctctagcct

SEQ ID NO: 326 - DNA, 30 bp, Artificial sequence
  transposase binding site
aggctagaggatgccttgtcacccgttaag

SEQ ID NO: 327 - DNA, 30 bp, Artificial sequence
  transposase binding site
cttaacgggtgacaacgtagcctacgaagc

SEQ ID NO: 328 - DNA, 30 bp, Artificial sequence
  transposase binding site
gcttcgtaggctacgttgtcacccgttaag

SEQ ID NO: 329 - DNA, 29 bp, Artificial sequence
  transposase binding site
ccttaattccgcaacactatagtttaaca

SEQ ID NO: 330 - DNA, 29 bp, Artificial sequence
  transposase binding site
tgttaaactatagtgttgcggaattaagg

SEQ ID NO: 331 - DNA, 29 bp, Artificial sequence
  transposase binding site
cctcaaatccgcaacctatagggtttagt

SEQ ID NO: 332 - DNA, 29 bp, Artificial sequence
  transposase binding site
actaaaccctataggttgcggatttgagg

SEQ ID NO: 333 - DNA, 29 bp, Artificial sequence
  transposase binding site
cagtacctcacaaagccggttagttgaga

SEQ ID NO: 334 - DNA, 29 bp, Artificial sequence
  transposase binding site
tctcaactaaccggctttgtgaggtactg

SEQ ID NO: 335 - DNA, 29 bp, Artificial sequence
  transposase binding site
cagtacctcacaaagcattctcggctagc

SEQ ID NO: 336 - DNA, 29 bp, Artificial sequence
  transposase binding site
gctagccgagaatgctttgtgaggtactg

SEQ ID NO: 337 - DNA, 37 bp, Artificial sequence
  transposase binding site
ggccgtgaacccataaactgggtaccggattactgat

SEQ ID NO: 338 - DNA, 37 bp, Artificial sequence
  transposase binding site
atcagtaatccggtacccagtttatgggttcacggcc

SEQ ID NO: 339 - DNA, 37 bp, Artificial sequence
  transposase binding site
ggccgtagactcataagcccgcagccacaggcgcatt

SEQ ID NO: 340 - DNA, 37 bp, Artificial sequence
  transposase binding site
aatgcgcctgtggctgcgggcttatgagtctacggcc

SEQ ID NO: 341 - DNA, 37 bp, Artificial sequence
  transposase binding site
gggcttgtctgcattcaaggattcccttttgtacgaa

SEQ ID NO: 342 - DNA, 37 bp, Artificial sequence
  transposase binding site
ttcgtacaaaagggaatccttgaatgcagacaagccc

SEQ ID NO: 343 - DNA, 37 bp, Artificial sequence
  transposase binding site
gggcgtgtctgcattcaacgtaaccagatcatagcgc

SEQ ID NO: 344 - DNA, 37 bp, Artificial sequence
  transposase binding site
gcgctatgatctggttacgttgaatgcagacacgccc

SEQ ID NO: 345 - DNA, 37 bp, Artificial sequence
  transposase binding site
ggctttgttgaataaatcgaacttttgctgagttgaa

SEQ ID NO: 346 - DNA, 37 bp, Artificial sequence
  transposase binding site
ttcaactcagcaaaagttcgatttattcaacaaagcc

SEQ ID NO: 347 - DNA, 37 bp, Artificial sequence
  transposase binding site
ggctttgttgaataaatcagatttcgggtaagtctcc

SEQ ID NO: 348 - DNA, 37 bp, Artificial sequence
  transposase binding site
ggagacttacccgaaatctgatttattcaacaaagcc

SEQ ID NO: 349 - DNA, 28 bp, Artificial sequence
  transposase binding site
ggtgatgctgccaacttactgatttagt

SEQ ID NO: 350 - DNA, 28 bp, Artificial sequence
  transposase binding site
actaaatcagtaagttggcagcatcacc

SEQ ID NO: 351 - DNA, 28 bp, Artificial sequence
  transposase binding site
ggtaatgactccaacttattgatagtgt

SEQ ID NO: 352 - DNA, 28 bp, Artificial sequence
  transposase binding site
acactatcaataagttggagtcattacc

SEQ ID NO: 353 - DNA, 28 bp, Artificial sequence
  transposase binding site
ggtgatgcctctaattagttgaatctga

SEQ ID NO: 354 - DNA, 28 bp, Artificial sequence
  transposase binding site
tcagattcaactaattagaggcatcacc

SEQ ID NO: 355 - DNA, 28 bp, Artificial sequence
  transposase binding site
ggtgatgcttccaattagtagaacatgt

SEQ ID NO: 356 - DNA, 28 bp, Artificial sequence
  transposase binding site
acatgttctactaattggaagcatcacc

SEQ ID NO: 357 - DNA, 28 bp, Artificial sequence
  transposase binding site
ggtcatgcattcaatgcggagcggagat

SEQ ID NO: 358 - DNA, 28 bp, Artificial sequence
  transposase binding site
atctccgctccgcattgaatgcatgacc

SEQ ID NO: 359 - DNA, 28 bp, Artificial sequence
  transposase binding site
ggtcatgtattcaatctggttattagta

SEQ ID NO: 360 - DNA, 28 bp, Artificial sequence
  transposase binding site
tactaataaccagattgaatacatgacc

SEQ ID NO: 361 - DNA, 28 bp, Artificial sequence
  transposase binding site
gagagtttcaaatagataatgatgtggg

SEQ ID NO: 362 - DNA, 28 bp, Artificial sequence
  transposase binding site
cccacatcattatctatttgaaactctc

SEQ ID NO: 363 - DNA, 28 bp, Artificial sequence
  transposase binding site
gagagtttcaagaaagtaatgagaggcg

SEQ ID NO: 364 - DNA, 28 bp, Artificial sequence
  transposase binding site
cgcctctcattactttcttgaaactctc

SEQ ID NO: 365 - DNA, 28 bp, Artificial sequence
  transposase binding site
ggcattggtagttaattatagttatata

SEQ ID NO: 366 - DNA, 28 bp, Artificial sequence
  transposase binding site
tatataactataattaactaccaatgcc

SEQ ID NO: 367 - DNA, 28 bp, Artificial sequence
  transposase binding site
ggtattgttaattaaatatagataactc

SEQ ID NO: 368 - DNA, 28 bp, Artificial sequence
  transposase binding site
gagttatctatatttaattaacaatacc

SEQ ID NO: 369 - DNA, 28 bp, Artificial sequence
  transposase binding site
gatagtgccgtcattaagctatttatat

SEQ ID NO: 370 - DNA, 28 bp, Artificial sequence
  transposase binding site
atataaatagcttaatgacggcactatc

SEQ ID NO: 371 - DNA, 28 bp, Artificial sequence
  transposase binding site
gatagtgtcgtcattaagctacaaattc

SEQ ID NO: 372 - DNA, 28 bp, Artificial sequence
  transposase binding site
gaatttgtagcttaatgacgacactatc

SEQ ID NO: 373 - DNA, 55 bp, Artificial sequence
  transposase binding site
  misc_feature (23)..(46): n is a, c, g, or t
gggagtgttctcatgcagtcatnnnnnnnnnnnnnnnnnnnnnnnnttatattag

SEQ ID NO: 374 - DNA, 55 bp, Artificial sequence
  transposase binding site
  misc_feature (10)..(33): n is a, c, g, or t
ctaatataannnnnnnnnnnnnnnnnnnnnnnnatgactgcatgagaacactccc

SEQ ID NO: 375 - DNA, 55 bp, Artificial sequence
  transposase binding site
  misc_feature (23)..(46): n is a, c, g, or t
gggagtgttctcatgcagtcatnnnnnnnnnnnnnnnnnnnnnnnnatattaagg

SEQ ID NO: 376 - DNA, 55 bp, Artificial sequence
  transposase binding site
  misc_feature (10)..(33): n is a, c, g, or t
ccttaatatnnnnnnnnnnnnnnnnnnnnnnnnatgactgcatgagaacactccc

SEQ ID NO: 377 - DNA, 49 bp, Artificial sequence
  transposase binding site
  misc_feature (23)..(40): n is a, c, g, or t
gggactgttctcaaacagtcatnnnnnnnnnnnnnnnnnngtaatatta

SEQ ID NO: 378 - DNA, 49 bp, Artificial sequence
  transposase binding site
  misc_feature (10)..(27): n is a, c, g, or t
taatattacnnnnnnnnnnnnnnnnnnatgactgtttgagaacagtccc

SEQ ID NO: 379 - DNA, 49 bp, Artificial sequence
  transposase binding site
  misc_feature (23)..(40): n is a, c, g, or t
gggactgttctcaaacagtcatnnnnnnnnnnnnnnnnnngtaaaaata

SEQ ID NO: 380 - DNA, 49 bp, Artificial sequence
  transposase binding site
  misc_feature (10)..(27): n is a, c, g, or t
tatttttacnnnnnnnnnnnnnnnnnnatgactgtttgagaacagtccc

SEQ ID NO: 381 - DNA, 54 bp, Artificial sequence
  transposase binding site
cagtgctggccaaaaagatatccacttttggttttttgtgtgtaacttttttct

SEQ ID NO: 382 - DNA, 54 bp, Artificial sequence
  transposase binding site
agaaaaaagttacacacaaaaaaccaaaagtggatatctttttggccagcactg

SEQ ID NO: 383 - DNA, 54 bp, Artificial sequence
  transposase binding site
gtcacgaccggtttttctataggtgaaaaccaaaaaacacacattgaaaaaaga

SEQ ID NO: 384 - DNA, 54 bp, Artificial sequence
  transposase binding site
tcttttttcaatgtgtgttttttggttttcacctatagaaaaaccggtcgtgac

SEQ ID NO: 385 - DNA, 32 bp, Artificial sequence
  transposase binding site
  misc_feature (1)..(1): N=T
  misc_feature (1)..(1): N= C ou A
  misc_feature (2)..(2): N=A
nngttgaagtcggaagtttacatacacttaag

SEQ ID NO: 386 - DNA, 32 bp, Artificial sequence
  transposase binding site
  misc_feature (31)..(31): N=T
  misc_feature (32)..(32): N=G ou A
cttaagtgtatgtaaacttccgacttcaacnn

SEQ ID NO: 387 - DNA, 32 bp, Artificial sequence
  transposase binding site
  misc_feature (1)..(1): N = T ou C
  misc_feature (2)..(2): N = A
nngttgaagtcggaagtttacatacaccttag

SEQ ID NO: 388 - DNA, 32 bp, Artificial sequence
  transposase binding site
  misc_feature (31)..(31): N= T
  misc_feature (32)..(32): N= G ou A
ctaaggtgtatgtaaacttccgacttcaacnn

SEQ ID NO: 389 - DNA, 22 bp, Artificial sequence
  transposase binding site
ctttcgcgtttttcgtgcgccg

SEQ ID NO: 390 - DNA, 22 bp, Artificial sequence
  transposase binding site
cggcgcacgaaaaacgcgaaag

SEQ ID NO: 391 - DNA, 22 bp, Artificial sequence
  transposase binding site
ttttcgcatttatcgtgaaacg

SEQ ID NO: 392 - DNA, 22 bp, Artificial sequence
  transposase binding site
cgtttcacgataaatgcgaaaa

SEQ ID NO: 393 - DNA, 22 bp, Artificial sequence
  transposase binding site
ctttcgcgtttttcgtgcgccg

SEQ ID NO: 394 - DNA, 22 bp, Artificial sequence
  transposase binding site
cggcgcacgaaaaacgcgaaag

SEQ ID NO: 395 - DNA, 23 bp, Artificial sequence
  transposase binding site
gttttcgcatttatcgtgaaacg

SEQ ID NO: 396 - DNA, 23 bp, Artificial sequence
  transposase binding site
cgtttcacgataaatgcgaaaac

SEQ ID NO: 397 - DNA, 22 bp, Artificial sequence
  transposase binding site
ctttcgcgtttttcgtgcgccg

SEQ ID NO: 398 - DNA, 22 bp, Artificial sequence
  transposase binding site
cggcgcacgaaaaacgcgaaag

SEQ ID NO: 399 - DNA, 22 bp, Artificial sequence
  transposase binding site
ttttcgcatttatcgtgaaacg

SEQ ID NO: 400 - DNA, 22 bp, Artificial sequence
  transposase binding site
cgtttcacgataaatgcgaaaa

SEQ ID NO: 401 - DNA, 38 bp, Artificial sequence
  transposase binding site
gaaagcgcaaaaagcacgcggcgcaaaaagcacgcggc

SEQ ID NO: 402 - DNA, 44 bp, Artificial sequence
  transposase binding site
gccgcgtgctttttgcgctttcgccgcgtgctttttgcgctttc

SEQ ID NO: 403 - DNA, 22 bp, Artificial sequence
  transposase binding site
ctttcgcgtttttcgtgcgccg

SEQ ID NO: 404 - DNA, 22 bp, Artificial sequence
  transposase binding site
cggcgcacgaaaaacgcgaaag

SEQ ID NO: 405 - DNA, 41 bp, Artificial sequence
  transposase binding site
tgtggggggacaaaaaagtctcaaactggacaaaaaagatc

SEQ ID NO: 406 - DNA, 41 bp, Artificial sequence
  transposase binding site
gatcttttttgtccagtttgagacttttttgtccgcccaca

SEQ ID NO: 407 - DNA, 41 bp, Artificial sequence
  transposase binding site
gatctattttgttcagttcaagactttattgtccgcccaca

SEQ ID NO: 408 - DNA, 41 bp, Artificial sequence
  transposase binding site
tgtgggcggacaataaagtcttgaactgaacaaaatagatc

SEQ ID NO: 409 - DNA, 50 bp, Artificial sequence
  transposase binding site
ggggtttggggagcaacggaaccaaaaaccaacgtaaggcttagctagag

SEQ ID NO: 410 - DNA, 50 bp, Artificial sequence
  transposase binding site
ctctagctaagccttacgttggtttttggttccgttgctccccaaacccc

SEQ ID NO: 411 - DNA, 50 bp, Artificial sequence
  transposase binding site
ggggtttggggagcaacggaacagaaagtgcacttaagcccagcgcctgc

SEQ ID NO: 412 - DNA, 50 bp, Artificial sequence
  transposase binding site
gcaggcgctgggcttaagtgcactttctgttccgttgctccccaaacccc

SEQ ID NO: 413 - DNA, 50 bp, Artificial sequence
  transposase binding site
ggggtttggggagcaacggaaccaaaaaccaacttaaggcttagctagag

SEQ ID NO: 414 - DNA, 50 bp, Artificial sequence
  transposase binding site
ctctagctaagccttaagttggtttttggttccgttgctccccaaacccc

SEQ ID NO: 415 - DNA, 50 bp, Artificial sequence; identical to SEQ ID NO: 411
  transposase binding site

SEQ ID NO: 416 - DNA, 50 bp, Artificial sequence; identical to SEQ ID NO: 412
  transposase binding site

SEQ ID NO: 417 - DNA, 50 bp, Artificial sequence
  transposase binding site
ggggtttggggagcaacggaaccaaaaaccaacgtaaggcttaccaacgc

SEQ ID NO: 418 - DNA, 50 bp, Artificial sequence
  transposase binding site
gcgttggtaagccttacgttggtttttggttccgttgctccccaaacccc

SEQ ID NO: 419 - DNA, 49 bp, Artificial sequence
  transposase binding site
ggggtttggggagcaatggaaccaaaaaccaacgtaagctctgaatccc

SEQ ID NO: 420 - DNA, 49 bp, Artificial sequence
  transposase binding site
gggattcagagcttacgttggtttttggttccattgctccccaaacccc

SEQ ID NO: 421 - DNA, 50 bp, Artificial sequence
  transposase binding site
ggggtttggggagcaacggaaccaaaaaccaacgtaaggcttaccacctg

SEQ ID NO: 422 - DNA, 50 bp, Artificial sequence
  transposase binding site
caggtggtaagccttacgttggtttttggttccgttgctccccaaacccc

SEQ ID NO: 423 - DNA, 49 bp, Artificial sequence
  transposase binding site
ggggtttggggagcaaggaaccaaaaaccaacgtaagccctaccagcgc

SEQ ID NO: 424 - DNA, 49 bp, Artificial sequence
  transposase binding site
gcgctggtagggcttacgttggtttttggttccttgctccccaaacccc

SEQ ID NO: 425 - DNA, 9 bp, Artificial sequence
  domaine riche en G/C
ggcgatcgc

SEQ ID NO: 426 - DNA, 12 bp, Artificial sequence
  domaine riche en G/C
gcggcgatcggc

SEQ ID NO: 427 - DNA, 6 bp, Artificial sequence
  domaine riche en G/C
ggtcgc

SEQ ID NO: 428 - DNA, 6 bp, Artificial sequence
  domaine riche en G/C
gcgacc

SEQ ID NO: 429 - DNA, 798 bp, Artificial sequence
  sequence de la figure 12
  misc_feature (1)..(29): n is a, c, g, or t
  misc_feature (40)..(40): n is a, c, g, or t
  misc_feature (78)..(88): n is a, c, g, or t
  misc_feature (214)..(215): n is a, c, g, or t
  misc_feature (218)..(219): n is a, c, g, or t
  misc_feature (225)..(226): n is a, c, g, or t
  misc_feature (228)..(228): n is a, c, g, or t
  misc_feature (230)..(230): n is a, c, g, or t
  misc_feature (232)..(232): n is a, c, g, or t
  misc_feature (236)..(237): n is a, c, g, or t
  misc_feature (240)..(240): n is a, c, g, or t
  misc_feature (243)..(243): n is a, c, g, or t
  misc_feature (248)..(248): n is a, c, g, or t
  misc_feature (250)..(251): n is a, c, g, or t
  misc_feature (254)..(254): n is a, c, g, or t
  misc_feature (257)..(259): n is a, c, g, or t
  misc_feature (264)..(264): n is a, c, g, or t
  misc_feature (266)..(267): n is a, c, g, or t
  misc_feature (269)..(269): n is a, c, g, or t
  misc_feature (271)..(271): n is a, c, g, or t
  misc_feature (274)..(274): n is a, c, g, or t
  misc_feature (276)..(281): n is a, c, g, or t
  misc_feature (284)..(284): n is a, c, g, or t
  misc_feature (317)..(317): n is a, c, g, or t
  misc_feature (323)..(323): n is a, c, g, or t
  misc_feature (325)..(327): n is a, c, g, or t
  misc_feature (329)..(329): n is a, c, g, or t
  misc_feature (339)..(339): n is a, c, g, or t
  misc_feature (341)..(341): n is a, c, g, or t
  misc_feature (343)..(343): n is a, c, g, or t
  misc_feature (351)..(352): n is a, c, g, or t
  misc_feature (357)..(357): n is a, c, g, or t
  misc_feature (359)..(359): n is a, c, g, or t
  misc_feature (364)..(364): n is a, c, g, or t
  misc_feature (374)..(375): n is a, c, g, or t
  misc_feature (381)..(381): n is a, c, g, or t
  misc_feature (383)..(383): n is a, c, g, or t
  misc_feature (386)..(387): n is a, c, g, or t
  misc_feature (389)..(389): n is a, c, g, or t
  misc_feature (392)..(394): n is a, c, g, or t
  misc_feature (399)..(399): n is a, c, g, or t
  misc_feature (401)..(404): n is a, c, g, or t
  misc_feature (686)..(687): n is a, c, g, or t
  misc_feature (728)..(728): n is a, c, g, or t
  misc_feature (738)..(739): n is a, c, g, or t
  misc_feature (753)..(753): n is a, c, g, or t
  misc_feature (768)..(769): n is a, c, g, or t
  misc_feature (787)..(787): n is a, c, g, or t
  misc_feature (794)..(794): n is a, c, g, or t
nnnnnnnnnnnnnnnnnnnnnnnnnnnnnagctcgccgancactaccagcagaacacccccaccatgttatcctcctnnnnnnnnnnncgacaaccactacctgagcacccagtccgccctgagcaaagaccccaacgagaagcgcgatcacatggtcctgctggagttcgtgaccgccgccgggatcactctcggcatggacgagctgtacanntcnncaatgnnancngnggannggnggncctcngnncgntcnnnctgtncnncnanggngnnnnnntcnttgtgggaggtgatgtccaacttgatgttgacnttgtangnnncnggcagctgcncngncttcttgnncttgnangtggncttgacctcnncgtcgnanggnncnccnnncttcntnnnnagcctctgcttgatctcgcccttcagggcgccgtcctcggggtacatccgctcggaggaggcctcccagcccatggtcttcttctgcattacggggccgtcggaggggaagttggtgccgcgcagcttcaccttgtagatgaactcgccgtcctgcagggaggagtcctgggtcacggtcaccacgccgccgtcctcgaagttcatcacgcgctcccacttgaagccctcggggaaggacagcttcaagtagtcggggatgtcggcggggtgcttcacgtannccttggagccgtacatgaactgaggggacaggatgtcccangcgaagggcnngggccacccttggncaccttcagcttggnngtctgggtgccctcgtangggcggncctc

SEQ ID NO: 430 - DNA, 392 bp, Artificial sequence
  sequence de la figure 14
  misc_feature (1)..(19): n is a, c, g, or t
  misc_feature (22)..(22): n is a, c, g, or t
  misc_feature (24)..(24): n is a, c, g, or t
  misc_feature (26)..(27): n is a, c, g, or t
  misc_feature (30)..(34): n is a, c, g, or t
  misc_feature (38)..(38): n is a, c, g, or t
  misc_feature (143)..(152): n is a, c, g, or t
  misc_feature (154)..(165): n is a, c, g, or t
  misc_feature (167)..(167): n is a, c, g, or t
  misc_feature (172)..(172): n is a, c, g, or t
  misc_feature (175)..(175): n is a, c, g, or t
  misc_feature (178)..(182): n is a, c, g, or t
  misc_feature (184)..(190): n is a, c, g, or t
  misc_feature (192)..(193): n is a, c, g, or t
  misc_feature (195)..(196): n is a, c, g, or t
  misc_feature (198)..(201): n is a, c, g, or t
  misc_feature (203)..(224): n is a, c, g, or t
  misc_feature (226)..(229): n is a, c, g, or t
  misc_feature (232)..(235): n is a, c, g, or t
  misc_feature (238)..(248): n is a, c, g, or t
  misc_feature (250)..(250): n is a, c, g, or t
  misc_feature (253)..(253): n is a, c, g, or t
  misc_feature (255)..(256): n is a, c, g, or t
  misc_feature (258)..(262): n is a, c, g, or t
  misc_feature (264)..(267): n is a, c, g, or t
  misc_feature (269)..(271): n is a, c, g, or t
  misc_feature (274)..(278): n is a, c, g, or t
  misc_feature (280)..(281): n is a, c, g, or t
  misc_feature (285)..(287): n is a, c, g, or t
  misc_feature (290)..(290): n is a, c, g, or t
  misc_feature (292)..(298): n is a, c, g, or t
  misc_feature (300)..(302): n is a, c, g, or t
  misc_feature (305)..(311): n is a, c, g, or t
  misc_feature (313)..(324): n is a, c, g, or t
  misc_feature (327)..(330): n is a, c, g, or t
  misc_feature (332)..(333): n is a, c, g, or t
  misc_feature (336)..(337): n is a, c, g, or t
  misc_feature (340)..(341): n is a, c, g, or t
  misc_feature (344)..(348): n is a, c, g, or t
  misc_feature (351)..(356): n is a, c, g, or t
  misc_feature (360)..(383): n is a, c, g, or t
  misc_feature (385)..(388): n is a, c, g, or t
  misc_feature (390)..(392): n is a, c, g, or t
nnnnnnnnnnnnnnnnnnngtnanannggnnnnntccncatcatcggcgcagtgggcatcggcattgccgtggtcatgatatttggcatgatcttcagtatgatcttgtgctgtgctatccgcaggaaccgcgagatggtcannnnnnnnnntnnnnnnnnnnnngngtganggncannnnnannnnnnnanngnnannnnannnnnnnnnnnnnnnnnnnnnncnnnnccnnnnccnnnnnnnnnnncntcntnnannnnncnnnntnnnttnnnnntnntccnnnacntnnnnnnncnnnttnnnnnnntnnnnnnnnnnnncannnncnncannttnntcnnnnnctnnnnnntccnnnnnnnnnnnnnnnnnnnnnnnnannnnannn

SEQ ID NO: 431 - DNA, 673 bp, Artificial sequence
  sequence de la figure 16
  misc_feature (1)..(10): n is a, c, g, or t
  misc_feature (15)..(19): n is a, c, g, or t
  misc_feature (24)..(24): n is a, c, g, or t
  misc_feature (34)..(34): n is a, c, g, or t
  misc_feature (60)..(60): n is a, c, g, or t
  misc_feature (63)..(63): n is a, c, g, or t
  misc_feature (71)..(73): n is a, c, g, or t
  misc_feature (107)..(107): n is a, c, g, or t
  misc_feature (170)..(170): n is a, c, g, or t
  misc_feature (186)..(188): n is a, c, g, or t
  misc_feature (252)..(252): n is a, c, g, or t
  misc_feature (259)..(259): n is a, c, g, or t
  misc_feature (268)..(268): n is a, c, g, or t
  misc_feature (288)..(291): n is a, c, g, or t
  misc_feature (338)..(339): n is a, c, g, or t
  misc_feature (341)..(341): n is a, c, g, or t
  misc_feature (346)..(347): n is a, c, g, or t
  misc_feature (359)..(362): n is a, c, g, or t
  misc_feature (364)..(364): n is a, c, g, or t
  misc_feature (366)..(367): n is a, c, g, or t
  misc_feature (370)..(370): n is a, c, g, or t
  misc_feature (373)..(373): n is a, c, g, or t
  misc_feature (376)..(376): n is a, c, g, or t
  misc_feature (378)..(382): n is a, c, g, or t
  misc_feature (384)..(389): n is a, c, g, or t
  misc_feature (393)..(394): n is a, c, g, or t
  misc_feature (407)..(409): n is a, c, g, or t
  misc_feature (412)..(412): n is a, c, g, or t
  misc_feature (414)..(435): n is a, c, g, or t
  misc_feature (437)..(439): n is a, c, g, or t
  misc_feature (442)..(443): n is a, c, g, or t
  misc_feature (445)..(445): n is a, c, g, or t
  misc_feature (447)..(448): n is a, c, g, or t
  misc_feature (450)..(450): n is a, c, g, or t
  misc_feature (452)..(458): n is a, c, g, or t
  misc_feature (466)..(466): n is a, c, g, or t
  misc_feature (470)..(470): n is a, c, g, or t
  misc_feature (473)..(474): n is a, c, g, or t
  misc_feature (482)..(486): n is a, c, g, or t
  misc_feature (488)..(490): n is a, c, g, or t
  misc_feature (495)..(508): n is a, c, g, or t
  misc_feature (510)..(512): n is a, c, g, or t
  misc_feature (514)..(514): n is a, c, g, or t
  misc_feature (516)..(532): n is a, c, g, or t
  misc_feature (534)..(539): n is a, c, g, or t
  misc_feature (541)..(559): n is a, c, g, or t
  misc_feature (561)..(562): n is a, c, g, or t
  misc_feature (564)..(568): n is a, c, g, or t
  misc_feature (572)..(595): n is a, c, g, or t
  misc_feature (597)..(599): n is a, c, g, or t
  misc_feature (606)..(609): n is a, c, g, or t
  misc_feature (611)..(611): n is a, c, g, or t
  misc_feature (613)..(617): n is a, c, g, or t
  misc_feature (619)..(633): n is a, c, g, or t
  misc_feature (635)..(635): n is a, c, g, or t
  misc_feature (638)..(664): n is a, c, g, or t
  misc_feature (666)..(673): n is a, c, g, or t
nnnnnnnnnnctgannnnntgccnaatatcatgnccacggcaatgccgatgcccactgcnccnatgatgtnnnaatttattgtcgaagacctctttgatggcatcangacaggacttcacggtgaaggtttcgagtacgtccttcttggggcagatgtctgagataaacngctcctcgcccttgannnaaccacagcagttcaacgcatagtggatggctttcagcgtttcccgctggggctcattgaacanctcctcncccttgaangtgtccttgtaaaactcctnnnnttccttaatcacctcatccttgtgggaatatccccagatggccgcanntngatcnntggcgaatatcnnnnanannaanccnaanannnnnannnnnntgcnntgggactcctgcnnnccngnnnnnnnnnnnnnnnnnnnnnngnnntannangnnanannnnnnnatcctacntttnacnnccctaccnnnnngnnnaattnnnnnnnnnnnnnncnnncncnnnnnnnnnnnnnnnnncnnnnnncnnnnnnnnnnnnnnnnnnntnncnnnnncccnnnnnnnnnnnnnnnnnnnnnnnncnnnccccacnnnnangnnnnnannnnnnnnnnnnnnncnctnnnnnnnnnnnnnnnnnnnnnnnnnnntnnnnnnnn

SEQ ID NO: 432 - DNA, 671 bp, Artificial sequence
  sequence de la figure 19
  misc_feature (1)..(10): n is a, c, g, or t
  misc_feature (12)..(24): n is a, c, g, or t
  misc_feature (27)..(28): n is a, c, g, or t
  misc_feature (30)..(38): n is a, c, g, or t
  misc_feature (40)..(42): n is a, c, g, or t
  misc_feature (46)..(51): n is a, c, g, or t
  misc_feature (53)..(54): n is a, c, g, or t
  misc_feature (56)..(61): n is a, c, g, or t
  misc_feature (63)..(64): n is a, c, g, or t
  misc_feature (66)..(69): n is a, c, g, or t
  misc_feature (71)..(71): n is a, c, g, or t
  misc_feature (75)..(75): n is a, c, g, or t
  misc_feature (77)..(79): n is a, c, g, or t
  misc_feature (81)..(84): n is a, c, g, or t
  misc_feature (87)..(87): n is a, c, g, or t
  misc_feature (93)..(93): n is a, c, g, or t
  misc_feature (95)..(96): n is a, c, g, or t
  misc_feature (98)..(98): n is a, c, g, or t
  misc_feature (102)..(103): n is a, c, g, or t
  misc_feature (108)..(109): n is a, c, g, or t
  misc_feature (112)..(114): n is a, c, g, or t
  misc_feature (116)..(117): n is a, c, g, or t
  misc_feature (120)..(120): n is a, c, g, or t
  misc_feature (122)..(122): n is a, c, g, or t
  misc_feature (126)..(126): n is a, c, g, or t
  misc_feature (132)..(132): n is a, c, g, or t
  misc_feature (135)..(135): n is a, c, g, or t
  misc_feature (137)..(137): n is a, c, g, or t
  misc_feature (141)..(141): n is a, c, g, or t
  misc_feature (150)..(150): n is a, c, g, or t
  misc_feature (152)..(152): n is a, c, g, or t
  misc_feature (159)..(159): n is a, c, g, or t
  misc_feature (163)..(167): n is a, c, g, or t
  misc_feature (170)..(171): n is a, c, g, or t
  misc_feature (181)..(182): n is a, c, g, or t
  misc_feature (186)..(186): n is a, c, g, or t
  misc_feature (189)..(189): n is a, c, g, or t
  misc_feature (195)..(195): n is a, c, g, or t
  misc_feature (198)..(198): n is a, c, g, or t
  misc_feature (203)..(204): n is a, c, g, or t
  misc_feature (209)..(209): n is a, c, g, or t
  misc_feature (212)..(212): n is a, c, g, or t
  misc_feature (228)..(230): n is a, c, g, or t
  misc_feature (234)..(234): n is a, c, g, or t
  misc_feature (240)..(240): n is a, c, g, or t
  misc_feature (246)..(248): n is a, c, g, or t
  misc_feature (253)..(253): n is a, c, g, or t
  misc_feature (266)..(266): n is a, c, g, or t
  misc_feature (270)..(270): n is a, c, g, or t
  misc_feature (276)..(276): n is a, c, g, or t
  misc_feature (279)..(279): n is a, c, g, or t
  misc_feature (285)..(288): n is a, c, g, or t
  misc_feature (290)..(290): n is a, c, g, or t
  misc_feature (292)..(292): n is a, c, g, or t
  misc_feature (294)..(294): n is a, c, g, or t
  misc_feature (297)..(297): n is a, c, g, or t
  misc_feature (305)..(305): n is a, c, g, or t
  misc_feature (312)..(312): n is a, c, g, or t
  misc_feature (318)..(320): n is a, c, g, or t
  misc_feature (363)..(367): n is a, c, g, or t
  misc_feature (370)..(370): n is a, c, g, or t
  misc_feature (378)..(381): n is a, c, g, or t
  misc_feature (394)..(398): n is a, c, g, or t
  misc_feature (400)..(401): n is a, c, g, or t
  misc_feature (408)..(408): n is a, c, g, or t
  misc_feature (411)..(412): n is a, c, g, or t
  misc_feature (419)..(419): n is a, c, g, or t
  misc_feature (423)..(423): n is a, c, g, or t
  misc_feature (430)..(430): n is a, c, g, or t
  misc_feature (433)..(433): n is a, c, g, or t
  misc_feature (435)..(436): n is a, c, g, or t
  misc_feature (438)..(438): n is a, c, g, or t
  misc_feature (441)..(441): n is a, c, g, or t
  misc_feature (443)..(443): n is a, c, g, or t
  misc_feature (447)..(447): n is a, c, g, or t
  misc_feature (449)..(449): n is a, c, g, or t
  misc_feature (451)..(451): n is a, c, g, or t
  misc_feature (453)..(464): n is a, c, g, or t
  misc_feature (467)..(472): n is a, c, g, or t
  misc_feature (476)..(476): n is a, c, g, or t
  misc_feature (478)..(479): n is a, c, g, or t
  misc_feature (481)..(481): n is a, c, g, or t
  misc_feature (483)..(484): n is a, c, g, or t
  misc_feature (487)..(489): n is a, c, g, or t
  misc_feature (491)..(491): n is a, c, g, or t
  misc_feature (493)..(497): n is a, c, g, or t
  misc_feature (500)..(502): n is a, c, g, or t
  misc_feature (505)..(511): n is a, c, g, or t
  misc_feature (513)..(513): n is a, c, g, or t
  misc_feature (515)..(517): n is a, c, g, or t
  misc_feature (519)..(523): n is a, c, g, or t
  misc_feature (525)..(526): n is a, c, g, or t
  misc_feature (528)..(544): n is a, c, g, or t
  misc_feature (546)..(549): n is a, c, g, or t
  misc_feature (552)..(553): n is a, c, g, or t
  misc_feature (555)..(555): n is a, c, g, or t
  misc_feature (557)..(571): n is a, c, g, or t
  misc_feature (574)..(584): n is a, c, g, or t
  misc_feature (586)..(589): n is a, c, g, or t
  misc_feature (591)..(594): n is a, c, g, or t
  misc_feature (597)..(606): n is a, c, g, or t
  misc_feature (609)..(610): n is a, c, g, or t
  misc_feature (612)..(617): n is a, c, g, or t
  misc_feature (621)..(622): n is a, c, g, or t
  misc_feature (624)..(624): n is a, c, g, or t
  misc_feature (627)..(630): n is a, c, g, or t
  misc_feature (632)..(633): n is a, c, g, or t
  misc_feature (635)..(635): n is a, c, g, or t
  misc_feature (641)..(641): n is a, c, g, or t
  misc_feature (643)..(643): n is a, c, g, or t
  misc_feature (645)..(646): n is a, c, g, or t
  misc_feature (649)..(654): n is a, c, g, or t
  misc_feature (656)..(656): n is a, c, g, or t
  misc_feature (658)..(664): n is a, c, g, or t
  misc_feature (666)..(666): n is a, c, g, or t
  misc_feature (668)..(671): n is a, c, g, or t
nnnnnnnnnntnnnnnnnnnnnnnagnncnnnnnnnnngnnnctcnnnnnntnngnnnnnngnntnnnncngcantnnngnnnntgnccgtgncnngncccnncctcnngannncnntgncntacngcgtgnagngnttcngccgctacncntaccacntgannnnncannacttcttcanntccnccntgcccnaangctanntccangancgcaccatcttcttcnnngacnacggcnactacnnnacccncgccgaggtgaanttcnagggcnacnccctgnnnnancncntcnagctgaanggcatcnacttcnnngaggacggcaacatcctggggcacaagctggagtacaactacnnnnnccncaacgtcnnnntcatggccgactnnnnnannaacggcntcnnggtgaanttcnagatccnccncnncntcnangacngnancnnnnnnnnnnnngannnnnnccancnnancnnccnnntngnnnnnggnnnctnnnnnnntncnnnannnnnannannnnnnnnnnnnnnnnncnnnnaannanannnnnnnnnnnnnnnacnnnnnnnnnnncnnnntnnnnaannnnnnnnnnacnncnnnnnntccnntngannnntnnantgtatntnanngtnnnnnntntnnnnnnntntnnnn

SEQ ID NO: 433 - DNA, 812 bp, Artificial sequence
  sequence de la figure 19
atggtgagcaagggcgaggagctgttcaccggggtggtgcccatcctggtcgagctggacggcgacgtaaacggccacaagttcagcgtgtccggcgagggcgagggcgatgccacctacggcaagctgaccctgaagttcatctgcaccaccggcaagctgcccgtgccctggcccaccctcgtgaccaccctgacctacggcgtgcagtgcttcagccgctaccccgaccacatgaagcagcacgacttcttcaagtccgccatgcccgaaggctacgtccaggagcgcaccatcttcttcaaggacgacggcaactacaagacccgcgccgaggtgaagttcgagggcgacaccctggtgaaccgcatcgagctgaagggcatcgacttcaaggaggacggcaacatcctggggcacaagctggagtacaactacaacagccacaacgtctatatcatggccgacaagcagaagaacggcatcaaggtgaacttcaagatccgccacaacatcgaggacggcagcgtgcagctcgccgaccactaccagcagaacacccccatcggcgacggccccgtgctgctgcccgacaaccactacctgagcacccagtccgccctgagcaaagaccccaacgagaagcgcgatcacatggtcctgctggagttcgtgaccgccgccgggatcactctcggcatggacgagctgtacaagtccggataataattttttttttttttttttttttagatgtgtataagagacagctgggcacgcgtataagcagctgagatgtgtataagagacag

SEQ ID NO: 434 - DNA, 270 bp, Artificial sequence
  sequence de la figure 19
  misc_feature (4)..(4): n is a, c, g, or t
  misc_feature (10)..(10): n is a, c, g, or t
  misc_feature (13)..(13): n is a, c, g, or t
  misc_feature (15)..(15): n is a, c, g, or t
  misc_feature (19)..(19): n is a, c, g, or t
  misc_feature (28)..(28): n is a, c, g, or t
  misc_feature (30)..(30): n is a, c, g, or t
  misc_feature (37)..(37): n is a, c, g, or t
  misc_feature (41)..(45): n is a, c, g, or t
  misc_feature (48)..(49): n is a, c, g, or t
  misc_feature (59)..(60): n is a, c, g, or t
  misc_feature (64)..(64): n is a, c, g, or t
  misc_feature (67)..(67): n is a, c, g, or t
  misc_feature (73)..(73): n is a, c, g, or t
  misc_feature (76)..(76): n is a, c, g, or t
  misc_feature (81)..(82): n is a, c, g, or t
  misc_feature (87)..(87): n is a, c, g, or t
  misc_feature (90)..(90): n is a, c, g, or t
  misc_feature (106)..(108): n is a, c, g, or t
  misc_feature (112)..(112): n is a, c, g, or t
  misc_feature (118)..(118): n is a, c, g, or t
  misc_feature (124)..(126): n is a, c, g, or t
  misc_feature (131)..(131): n is a, c, g, or t
  misc_feature (144)..(144): n is a, c, g, or t
  misc_feature (148)..(148): n is a, c, g, or t
  misc_feature (154)..(154): n is a, c, g, or t
  misc_feature (157)..(157): n is a, c, g, or t
  misc_feature (163)..(166): n is a, c, g, or t
  misc_feature (168)..(168): n is a, c, g, or t
  misc_feature (170)..(170): n is a, c, g, or t
  misc_feature (172)..(172): n is a, c, g, or t
  misc_feature (175)..(175): n is a, c, g, or t
  misc_feature (183)..(183): n is a, c, g, or t
  misc_feature (190)..(190): n is a, c, g, or t
  misc_feature (196)..(198): n is a, c, g, or t
  misc_feature (241)..(245): n is a, c, g, or t
  misc_feature (248)..(248): n is a, c, g, or t
  misc_feature (256)..(259): n is a, c, g, or t
tacngcgtgnagngnttcngccgctacncntaccacntgannnnncannacttcttcanntccnccntgcccnaangctanntccangancgcaccatcttcttcnnngacnacggcnactacnnnacccncgccgaggtgaanttcnagggcnacnccctgnnnnancncntcnagctgaanggcatcnacttcnnngaggacggcaacatcctggggcacaagctggagtacaactacnnnnnccncaacgtcnnnntcatggccgac

SEQ ID NO: 435 - DNA, 270 bp, Artificial sequence
  sequence de la figure 19
tacggcgtgcagtgcttcagccgctaccccgaccacatgaagcagcacgacttcttcaagtccgccatgcccgaaggctacgtccaggagcgcaccatcttcttcaaggacgacggcaactacaagacccgcgccgaggtgaagttcgagggcgacaccctggtgaaccgcatcgagctgaagggcatcgacttcaaggaggacggcaacatcctggggcacaagctggagtacaactacaacagccacaacgtctatatcatggccgac

SEQ ID NO: 436 - DNA, 131 bp, Artificial sequence
  première mol cule du complexe
  misc_feature (9)..(9): site de liaison à la transposase
  misc_feature (66)..(66): s quence A permettant l'insertion d'une s quence compl mentaire d'un acide nucl ique d'int r t
  misc_feature (123)..(123): site de liaison à la transposase
tgcagctgntttttttttttttttttttttttttttggcgatcgcttttttttttttttttttttnttttttttttttttttttttgcgatcgccttttttttttttttttgatacatgtttnctgtaagc

SEQ ID NO: 437 - DNA, 59 bp, Artificial sequence
  deuxième mol cule du complexe
  misc_feature (1)..(1): site de liaison à la transposase
  misc_feature (24)..(24): site de liaison à la transposase
  misc_feature (59)..(59): replacement sequence
ncagctgcagacaaagcttacagnttttttttttttttttttttttcatatgccaagtn

SEQ ID NO: 438 - DNA, 167 bp, Artificial sequence; identical to SEQ ID NO: 7
  première mol cule du complexe
  misc_feature (84)..(84): s quence A permettant l'insertion d'une s quence compl mentaire d'un acide nucl ique d'int r t

SEQ ID NO: 439 - DNA, 95 bp, Artificial sequence; identical to SEQ ID NO: 8
  deuxième mol cule du complexe
  misc_feature (95)..(95): replacement sequence

SEQ ID NO: 440 - DNA, 125 bp, Artificial sequence
  molecule of the complex
  misc_feature (9)..(9): Site de liaison à la transposase
  misc_feature (63)..(63): s quence A permettant l'insertion d'une s quence compl mentaire d'un acide nucl ique d'int r t
  misc_feature (117)..(117): Site de liaison à la transposase
tgcagctgntttttttttttttttttttttttttttggtcgcttttttttttttttttttttnttttttttttttttttttttgcgaccttttttttttttttttgatacatgtttnctgtaagc

SEQ ID NO: 441 - DNA, 53 bp, Artificial sequence
  molecule of the complex
  misc_feature (1)..(1): Site de liaison à la transposase
  misc_feature (24)..(24): Site de liaison à la transposase
  misc_feature (47)..(47): replacement sequence
ncagctgcagacaaagcttacagnttttttttttttttttttttttnccaagt

SEQ ID NO: 442 - DNA, 53 bp, Artificial sequence
  molecule of the complex
  misc_feature (1)..(1): Site de liaison à la transposase
  misc_feature (24)..(24): Site de liaison à la transposase
  misc_feature (53)..(53): replacement sequence
ncagctgcagacaaagcttacagnttttttttttttttttttttttccaagtn

SEQ ID NO: 443 - DNA, 137 bp, Artificial sequence
  molecule of the complex
  misc_feature (9)..(9): Site de liaison à la transposase
  misc_feature (69)..(69): s quence A permettant l'insertion d'une s quence compl mentaire d'un acide nucl ique d'int r t
  misc_feature (129)..(129): Site de liaison à la transposase
tgcagctgntttttttttttttttttttttttttttgcggcgatcggcttttttttttttttttttttnttttttttttttttttttttgccgatcgccgcttttttttttttttttgatacatgtttnctgtaagc

SEQ ID NO: 444 - DNA, 125 bp, Artificial sequence
  molecule of the complex
  misc_feature (9)..(9): Site de liaison à la transposase
  misc_feature (63)..(63): s quence A permettant l'insertion d'une s quence compl mentaire d'un acide nucl ique d'int r t
  misc_feature (117)..(117): Site de liaison à la transposase
gtgcccagntttctcgatcattttttttttttttttggtcgcttttttttttttttttttttnttttttttttttttttttttgcgacctttttttttttttttttttttttttttnctgcttat

SEQ ID NO: 445 - DNA, 63 bp, Artificial sequence
  molecule of the complex
  misc_feature (1)..(1): replacement sequence
  misc_feature (42)..(42): Site de liaison à la transposase
  misc_feature (63)..(63): Site de liaison à la transposase
ntacaagtccggataataattttttttttttttttttttttnctgggcacgcgtataagcagn

SEQ ID NO: 446 - DNA, 57 bp, Artificial sequence
  molecule of the complex
  misc_feature (7)..(7): replacement sequence
  misc_feature (36)..(36): Site de liaison à la transposase
  misc_feature (57)..(57): Site de liaison à la transposase
tacaagntaataattttttttttttttttttttttnctgggcacgcgtataagcagn

SEQ ID NO: 447 - DNA, 57 bp, Artificial sequence
  molecule of the complex
  misc_feature (1)..(1): replacement sequence
  misc_feature (36)..(36): Site de liaison à la transposase
  misc_feature (57)..(57): Site de liaison à la transposase
ntacaagtaataattttttttttttttttttttttnctgggcacgcgtataagcagn

SEQ ID NO: 448 - DNA, 131 bp, Artificial sequence
  molecule of the complex
  misc_feature (9)..(9): Site de liaison à la transposase
  misc_feature (66)..(66): s quence A permettant l'insertion d'une s quence compl mentaire d'un acide nucl ique d'int r t
  misc_feature (123)..(123): Site de liaison à la transposase
gtgcccagntttctcgatcattttttttttttttttggcgatcgcttttttttttttttttttttnttttttttttttttttttttgcgatcgcctttttttttttttttttttttttttttnctgcttat

SEQ ID NO: 449 - DNA, 137 bp, Artificial sequence
  molecule of the complex
  misc_feature (9)..(9): Site de liaison à la transposase
  misc_feature (69)..(69): s quence A permettant l'insertion d'une s quence compl mentaire d'un acide nucl ique d'int r t
  misc_feature (129)..(129): Site de liaison à la transposase
gtgcccagntttctcgatcattttttttttttttttgcggcgatcggcttttttttttttttttttttnttttttttttttttttttttgccgatcgccgctttttttttttttttttttttttttttnctgcttat

SEQ ID NO: 450 - DNA, 129 bp, Artificial sequence
  molecule of the complex
  misc_feature (7)..(7): Site de liaison à la transposase
  misc_feature (33)..(33): Site de liaison à la transposase
  misc_feature (78)..(78): s quence A permettant l'insertion d'une s quence compl mentaire d'un acide nucl ique d'int r t
  misc_feature (123)..(123): Site de liaison à la transposase
atcatcntttttttttttttttttgatagtagnttttttttttttttttttttttggtcgcttttttttttttttttnttttttttttttttttgcgacctttttttttttttgatacatttngatgat

SEQ ID NO: 451 - DNA, 46 bp, Artificial sequence
  molecule of the complex
  misc_feature (1)..(1): replacement sequence
  misc_feature (38)..(38): Site de liaison à la transposase
nacttggttaattaattttttttttttttttttttttnctactatc

SEQ ID NO: 452 - DNA, 46 bp, Artificial sequence
  molecule of the complex
  misc_feature (7)..(7): replacement sequence
  misc_feature (38)..(38): Site de liaison à la transposase
acttggnttaattaattttttttttttttttttttttnctactatc

SEQ ID NO: 453 - DNA, 52 bp, Artificial sequence
  molecule of the complex
  misc_feature (1)..(1): replacement sequence
  misc_feature (44)..(44): Site de liaison à la transposase
nacttggcatatgttaattaattttttttttttttttttttttnctactatc

SEQ ID NO: 454 - DNA, 141 bp, Artificial sequence
  molecule of the complex
  misc_feature (7)..(7): Site de liaison à la transposase
  misc_feature (33)..(33): Site de liaison à la transposase
  misc_feature (84)..(84): s quence A permettant l'insertion d'une s quence compl mentaire d'un acide nucl ique d'int r t
  misc_feature (135)..(135): Site de liaison à la transposase
atcatcntttttttttttttttttgatagtagnttttttttttttttttttttttgcggcgatcggcttttttttttttttttnttttttttttttttttgccgatcgccgctttttttttttttgatacatttngatgat

SEQ ID NO: 455 - DNA, 135 bp, Artificial sequence
  molecule of the complex
  misc_feature (9)..(9): Site de liaison à la transposase
  misc_feature (57)..(57): s quence A permettant l'insertion d'une s quence compl mentaire d'un acide nucl ique d'int r t
  misc_feature (105)..(105): Site de liaison à la transposase
  misc_feature (135)..(135): Site de liaison à la transposase
gatagtagnttttttttttttttttttttttggcgatcgcttttttttttttttttnttttttttttttttttgcgatcgcctttttttttttttgatacatttngatgattttttttttttttttttatcatcn

SEQ ID NO: 456 - DNA, 129 bp, Artificial sequence
  molecule of the complex
  misc_feature (9)..(9): Site de liaison à la transposase
  misc_feature (54)..(54): s quence A permettant l'insertion d'une s quence compl mentaire d'un acide nucl ique d'int r t
  misc_feature (99)..(99): Site de liaison à la transposase
  misc_feature (129)..(129): Site de liaison à la transposase
gatagtagnttttttttttttttttttttttggtcgcttttttttttttttttnttttttttttttttttgcgacctttttttttttttgatacatttngatgattttttttttttttttttatcatcn

SEQ ID NO: 457 - DNA, 141 bp, Artificial sequence
  molecule of the complex
  misc_feature (9)..(9): Site de liaison à la transposase
  misc_feature (60)..(60): s quence A permettant l'insertion d'une s quence compl mentaire d'un acide nucl ique d'int r t
  misc_feature (111)..(111): Site de liaison à la transposase
  misc_feature (141)..(141): Site de liaison à la transposase
gatagtagnttttttttttttttttttttttgcggcgatcggcttttttttttttttttnttttttttttttttttgccgatcgccgctttttttttttttgatacatttngatgattttttttttttttttttatcatcn

SEQ ID NO: 458 - DNA, 138 bp, Artificial sequence
  molecule of the complex
  misc_feature (7)..(7): Site de liaison à la transposase
  misc_feature (56)..(56): s quence A permettant l'insertion d'une s quence compl mentaire d'un acide nucl ique d'int r t
  misc_feature (103)..(103): Site de liaison à la transposase
  misc_feature (132)..(132): Site de liaison à la transposase
cacgtgntttctcgatcattattattttttggcgatcgcttttttttttttttttnttttttttttttttttgcgatcgcctttttttttttttttttttttngacgaatattttttttttttttttttttncacgtg

SEQ ID NO: 459 - DNA, 45 bp, Artificial sequence
  molecule of the complex
  misc_feature (9)..(9): Site de liaison à la transposase
  misc_feature (45)..(45): replacement sequence
tattcgtcnttttttttttttttttttattaattattacttgtan

SEQ ID NO: 460 - DNA, 45 bp, Artificial sequence
  molecule of the complex
  misc_feature (9)..(9): Site de liaison à la transposase
  misc_feature (39)..(39): n is a, c, g, or t
  misc_feature (39)..(39): Site de liaison à la transposase
tattcgtcnttttttttttttttttttattaattattancttgta

SEQ ID NO: 461 - DNA, 51 bp, Artificial sequence
  molecule of the complex
  misc_feature (9)..(9): Site de liaison à la transposase
  misc_feature (51)..(51): replacement sequence
tattcgtcnttttttttttttttttttattaattattatccggacttgtan

SEQ ID NO: 462 - DNA, 132 bp, Artificial sequence
  molecule of the complex
  misc_feature (7)..(7): Site de liaison à la transposase
  misc_feature (53)..(53): s quence A permettant l'insertion d'une s quence compl mentaire d'un acide nucl ique d'int r t
  misc_feature (97)..(97): Site de liaison à la transposase
  misc_feature (126)..(126): Site de liaison à la transposase
cacgtgntttctcgatcattattattttttggtcgcttttttttttttttttnttttttttttttttttgcgacctttttttttttttttttttttngacgaatattttttttttttttttttttncacgtg

SEQ ID NO: 463 - DNA, 144 bp, Artificial sequence
  molecule of the complex
  misc_feature (7)..(7): Site de liaison à la transposase
  misc_feature (59)..(59): s quence A permettant l'insertion d'une s quence compl mentaire d'un acide nucl ique d'int r t
  misc_feature (109)..(109): Site de liaison à la transposase
  misc_feature (138)..(138): Site de liaison à la transposase
cacgtgntttctcgatcattattattttttgcggcgatcggcttttttttttttttttnttttttttttttttttgccgatcgccgctttttttttttttttttttttngacgaatattttttttttttttttttttncacgtg

SEQ ID NO: 464 - DNA, 138 bp, Artificial sequence
  molecule of the complex
  misc_feature (1)..(1): Site de liaison à la transposase
  misc_feature (34)..(34): Site de liaison à la transposase
  misc_feature (83)..(83): s quence A permettant l'insertion d'une s quence compl mentaire d'un acide nucl ique d'int r t
  misc_feature (130)..(130): Site de liaison à la transposase
ncacgtgttttttttttttttttttttcacgtgntttctcgatcattattattttttggcgatcgcttttttttttttttttnttttttttttttttttgcgatcgcctttttttttttttttttttttngacgaata

SEQ ID NO: 465 - DNA, 132 bp, Artificial sequence
  molecule of the complex
  misc_feature (1)..(1): Site de liaison à la transposase
  misc_feature (34)..(34): Site de liaison à la transposase
  misc_feature (80)..(80): s quence A permettant l'insertion d'une s quence compl mentaire d'un acide nucl ique d'int r t
  misc_feature (124)..(124): Site de liaison à la transposase
ncacgtgttttttttttttttttttttcacgtgntttctcgatcattattattttttggtcgcttttttttttttttttnttttttttttttttttgcgacctttttttttttttttttttttngacgaata

SEQ ID NO: 466 - DNA, 144 bp, Artificial sequence
  molecule of the complex
  misc_feature (1)..(1): Site de liaison à la transposase
  misc_feature (34)..(34): Site de liaison à la transposase
  misc_feature (86)..(86): s quence A permettant l'insertion d'une s quence compl mentaire d'un acide nucl ique d'int r t
  misc_feature (136)..(136): Site de liaison à la transposase
ncacgtgttttttttttttttttttttcacgtgntttctcgatcattattattttttgcggcgatcggcttttttttttttttttnttttttttttttttttgccgatcgccgctttttttttttttttttttttngacgaata

SEQ ID NO: 467 - DNA, 167 bp, Artificial sequence; identical to SEQ ID NO: 7
  molecule of the complex
  misc_feature (84)..(84): s quence A permettant l'insertion d'une s quence compl mentaire d'un acide nucl ique d'int r t

SEQ ID NO: 468 - DNA, 167 bp, Artificial sequence
  molecule of the complex
  misc_feature (84)..(84): s quence A permettant l'insertion d'une s quence compl mentaire d'un acide nucl ique d'int r t
tgcagctgagatgtgtataagagacagtttttttttttttttttttttttttttggcgatcgcttttttttttttttttttttnttttttttttttttttttttgcgatcgccttttttttttttttttgatacatgtttctgtctcttatacacatctctgtaagc

SEQ ID NO: 469 - DNA, 161 bp, Artificial sequence
  molecule of the complex
  misc_feature (81)..(81): s quence A permettant l'insertion d'une s quence compl mentaire d'un acide nucl ique d'int r t
tgcagctgctgtctcttatacacatcttttttttttttttttttttttttttttggtcgcttttttttttttttttttttnttttttttttttttttttttgcgaccttttttttttttttttgatacatgtttagatgtgtataagagacagctgtaagc

SEQ ID NO: 470 - DNA, 161 bp, Artificial sequence
  molecule of the complex
  misc_feature (81)..(81): s quence A permettant l'insertion d'une s quence compl mentaire d'un acide nucl ique d'int r t
tgcagctgagatgtgtataagagacagtttttttttttttttttttttttttttggtcgcttttttttttttttttttttnttttttttttttttttttttgcgaccttttttttttttttttgatacatgtttctgtctcttatacacatctctgtaagc

SEQ ID NO: 471 - DNA, 173 bp, Artificial sequence
  molecule of the complex
  misc_feature (87)..(87): s quence A permettant l'insertion d'une s quence compl mentaire d'un acide nucl ique d'int r t
tgcagctgctgtctcttatacacatcttttttttttttttttttttttttttttgcggcgatcggcttttttttttttttttttttnttttttttttttttttttttgccgatcgccgcttttttttttttttttgatacatgtttagatgtgtataagagacagctgtaagc

SEQ ID NO: 472 - DNA, 173 bp, Artificial sequence
  molecule of the complex
  misc_feature (87)..(87): s quence A permettant l'insertion d'une s quence compl mentaire d'un acide nucl ique d'int r t
tgcagctgagatgtgtataagagacagtttttttttttttttttttttttttttgcggcgatcggcttttttttttttttttttttnttttttttttttttttttttgccgatcgccgcttttttttttttttttgatacatgtttctgtctcttatacacatctctgtaagc

SEQ ID NO: 473 - DNA, 161 bp, Artificial sequence
  molecule of the complex
  misc_feature (81)..(81): s quence A permettant l'insertion d'une s quence compl mentaire d'un acide nucl ique d'int r t
gtgcccagctgtctcttatacacatcttttctcgatcattttttttttttttttggtcgcttttttttttttttttttttnttttttttttttttttttttgcgacctttttttttttttttttttttttttttagatgtgtataagagacagctgcttat

SEQ ID NO: 474 - DNA, 161 bp, Artificial sequence
  molecule of the complex
  misc_feature (81)..(81): s quence A permettant l'insertion d'une s quence compl mentaire d'un acide nucl ique d'int r t
gtgcccagagatgtgtataagagacagtttctcgatcattttttttttttttttggtcgcttttttttttttttttttttnttttttttttttttttttttgcgacctttttttttttttttttttttttttttctgtctcttatacacatctctgcttat

SEQ ID NO: 475 - DNA, 167 bp, Artificial sequence
  molecule of the complex
  misc_feature (84)..(84): s quence A permettant l'insertion d'une s quence compl mentaire d'un acide nucl ique d'int r t
gtgcccagctgtctcttatacacatcttttctcgatcattttttttttttttttggcgatcgcttttttttttttttttttttnttttttttttttttttttttgcgatcgcctttttttttttttttttttttttttttagatgtgtataagagacagctgcttat

SEQ ID NO: 476 - DNA, 167 bp, Artificial sequence
  molecule of the complex
  misc_feature (84)..(84): s quence A permettant l'insertion d'une s quence compl mentaire d'un acide nucl ique d'int r t
gtgcccagagatgtgtataagagacagtttctcgatcattttttttttttttttggcgatcgcttttttttttttttttttttnttttttttttttttttttttgcgatcgcctttttttttttttttttttttttttttctgtctcttatacacatctctgcttat

SEQ ID NO: 477 - DNA, 173 bp, Artificial sequence
  molecule of the complex
  misc_feature (87)..(87): s quence A permettant l'insertion d'une s quence compl mentaire d'un acide nucl ique d'int r t
gtgcccagctgtctcttatacacatcttttctcgatcattttttttttttttttgcggcgatcggcttttttttttttttttttttnttttttttttttttttttttgccgatcgccgctttttttttttttttttttttttttttagatgtgtataagagacagctgcttat

SEQ ID NO: 478 - DNA, 173 bp, Artificial sequence
  molecule of the complex
  misc_feature (87)..(87): s quence A permettant l'insertion d'une s quence compl mentaire d'un acide nucl ique d'int r t
gtgcccagagatgtgtataagagacagtttctcgatcattttttttttttttttgcggcgatcggcttttttttttttttttttttnttttttttttttttttttttgccgatcgccgctttttttttttttttttttttttttttctgtctcttatacacatctctgcttat

SEQ ID NO: 479 - DNA, 189 bp, Artificial sequence; identical to SEQ ID NO: 9
  molecule of the complex
  misc_feature (117)..(117): s quence A permettant l'insertion d'une s quence compl mentaire d'un acide nucl ique d'int r t

SEQ ID NO: 480 - DNA, 189 bp, Artificial sequence
  molecule of the complex
  misc_feature (117)..(117): s quence A permettant l'insertion d'une s quence compl mentaire d'un acide nucl ique d'int r t
atcatcagatgtgtataagagacagtttttttttttttttttgatagtagagatgtgtataagagacagttttttttttttttttttttttggcgatcgcttttttttttttttttnttttttttttttttttgcgatcgcctttttttttttttgatacatttctgtctcttatacacatctgatgat

SEQ ID NO: 481 - DNA, 183 bp, Artificial sequence
  molecule of the complex
  misc_feature (114)..(114): s quence A permettant l'insertion d'une s quence compl mentaire d'un acide nucl ique d'int r t
atcatcctgtctcttatacacatcttttttttttttttttttgatagtagctgtctcttatacacatctttttttttttttttttttttttggtcgcttttttttttttttttnttttttttttttttttgcgacctttttttttttttgatacatttagatgtgtataagagacaggatgat

SEQ ID NO: 482 - DNA, 183 bp, Artificial sequence
  molecule of the complex
  misc_feature (114)..(114): s quence A permettant l'insertion d'une s quence compl mentaire d'un acide nucl ique d'int r t
atcatcagatgtgtataagagacagtttttttttttttttttgatagtagagatgtgtataagagacagttttttttttttttttttttttggtcgcttttttttttttttttnttttttttttttttttgcgacctttttttttttttgatacatttctgtctcttatacacatctgatgat

SEQ ID NO: 483 - DNA, 195 bp, Artificial sequence
  molecule of the complex
  misc_feature (120)..(120): s quence A permettant l'insertion d'une s quence compl mentaire d'un acide nucl ique d'int r t
atcatcctgtctcttatacacatcttttttttttttttttttgatagtagctgtctcttatacacatctttttttttttttttttttttttgcggcgatcggcttttttttttttttttnttttttttttttttttgccgatcgccgctttttttttttttgatacatttagatgtgtataagagacaggatgat

SEQ ID NO: 484 - DNA, 195 bp, Artificial sequence
  molecule of the complex
  misc_feature (120)..(120): s quence A permettant l'insertion d'une s quence compl mentaire d'un acide nucl ique d'int r t
atcatcagatgtgtataagagacagtttttttttttttttttgatagtagagatgtgtataagagacagttttttttttttttttttttttgcggcgatcggcttttttttttttttttnttttttttttttttttgccgatcgccgctttttttttttttgatacatttctgtctcttatacacatctgatgat

SEQ ID NO: 485 - DNA, 189 bp, Artificial sequence
  molecule of the complex
  misc_feature (75)..(75): s quence A permettant l'insertion d'une s quence compl mentaire d'un acide nucl ique d'int r t
gatagtagctgtctcttatacacatctttttttttttttttttttttttggcgatcgcttttttttttttttttnttttttttttttttttgcgatcgcctttttttttttttgatacatttagatgtgtataagagacaggatgattttttttttttttttttatcatcctgtctcttatacacatct

SEQ ID NO: 486 - DNA, 189 bp, Artificial sequence
  molecule of the complex
  misc_feature (75)..(75): s quence A permettant l'insertion d'une s quence compl mentaire d'un acide nucl ique d'int r t
gatagtagagatgtgtataagagacagttttttttttttttttttttttggcgatcgcttttttttttttttttnttttttttttttttttgcgatcgcctttttttttttttgatacatttctgtctcttatacacatctgatgattttttttttttttttttatcatcagatgtgtataagagacag

SEQ ID NO: 487 - DNA, 183 bp, Artificial sequence
  molecule of the complex
  misc_feature (72)..(72): s quence A permettant l'insertion d'une s quence compl mentaire d'un acide nucl ique d'int r t
gatagtagctgtctcttatacacatctttttttttttttttttttttttggtcgcttttttttttttttttnttttttttttttttttgcgacctttttttttttttgatacatttagatgtgtataagagacaggatgattttttttttttttttttatcatcctgtctcttatacacatct

SEQ ID NO: 488 - DNA, 183 bp, Artificial sequence
  molecule of the complex
  misc_feature (72)..(72): s quence A permettant l'insertion d'une s quence compl mentaire d'un acide nucl ique d'int r t
gatagtagagatgtgtataagagacagttttttttttttttttttttttggtcgcttttttttttttttttnttttttttttttttttgcgacctttttttttttttgatacatttctgtctcttatacacatctgatgattttttttttttttttttatcatcagatgtgtataagagacag

SEQ ID NO: 489 - DNA, 195 bp, Artificial sequence
  molecule of the complex
  misc_feature (78)..(78): s quence A permettant l'insertion d'une s quence compl mentaire d'un acide nucl ique d'int r t
gatagtagctgtctcttatacacatctttttttttttttttttttttttgcggcgatcggcttttttttttttttttnttttttttttttttttgccgatcgccgctttttttttttttgatacatttagatgtgtataagagacaggatgattttttttttttttttttatcatcctgtctcttatacacatct

SEQ ID NO: 490 - DNA, 195 bp, Artificial sequence
  molecule of the complex
  misc_feature (78)..(78): s quence A permettant l'insertion d'une s quence compl mentaire d'un acide nucl ique d'int r t
gatagtagagatgtgtataagagacagttttttttttttttttttttttgcggcgatcggcttttttttttttttttnttttttttttttttttgccgatcgccgctttttttttttttgatacatttctgtctcttatacacatctgatgattttttttttttttttttatcatcagatgtgtataagagacag

SEQ ID NO: 491 - DNA, 192 bp, Artificial sequence
  molecule of the complex
  misc_feature (74)..(74): s quence A permettant l'insertion d'une s quence compl mentaire d'un acide nucl ique d'int r t
cacgtgctgtctcttatacacatcttttctcgatcattattattttttggcgatcgcttttttttttttttttnttttttttttttttttgcgatcgcctttttttttttttttttttttagatgtgtataagagacaggacgaatattttttttttttttttttttagatgtgtataagagacagcacgtg

SEQ ID NO: 492 - DNA, 192 bp, Artificial sequence
  molecule of the complex
  misc_feature (74)..(74): s quence A permettant l'insertion d'une s quence compl mentaire d'un acide nucl ique d'int r t
cacgtgagatgtgtataagagacagtttctcgatcattattattttttggcgatcgcttttttttttttttttnttttttttttttttttgcgatcgcctttttttttttttttttttttctgtctcttatacacatctgacgaatattttttttttttttttttttctgtctcttatacacatctcacgtg

SEQ ID NO: 493 - DNA, 186 bp, Artificial sequence
  molecule of the complex
  misc_feature (71)..(71): s quence A permettant l'insertion d'une s quence compl mentaire d'un acide nucl ique d'int r t
cacgtgctgtctcttatacacatcttttctcgatcattattattttttggtcgcttttttttttttttttnttttttttttttttttgcgacctttttttttttttttttttttagatgtgtataagagacaggacgaatattttttttttttttttttttagatgtgtataagagacagcacgtg

SEQ ID NO: 494 - DNA, 186 bp, Artificial sequence
  molecule of the complex
  misc_feature (71)..(71): s quence A permettant l'insertion d'une s quence compl mentaire d'un acide nucl ique d'int r t
cacgtgagatgtgtataagagacagtttctcgatcattattattttttggtcgcttttttttttttttttnttttttttttttttttgcgacctttttttttttttttttttttctgtctcttatacacatctgacgaatattttttttttttttttttttctgtctcttatacacatctcacgtg

SEQ ID NO: 495 - DNA, 198 bp, Artificial sequence
  molecule of the complex
  misc_feature (77)..(77): s quence A permettant l'insertion d'une s quence compl mentaire d'un acide nucl ique d'int r t
cacgtgctgtctcttatacacatcttttctcgatcattattattttttgcggcgatcggcttttttttttttttttnttttttttttttttttgccgatcgccgctttttttttttttttttttttagatgtgtataagagacaggacgaatattttttttttttttttttttagatgtgtataagagacagcacgtg

SEQ ID NO: 496 - DNA, 198 bp, Artificial sequence
  molecule of the complex
  misc_feature (77)..(77): s quence A permettant l'insertion d'une s quence compl mentaire d'un acide nucl ique d'int r t
cacgtgagatgtgtataagagacagtttctcgatcattattattttttgcggcgatcggcttttttttttttttttnttttttttttttttttgccgatcgccgctttttttttttttttttttttctgtctcttatacacatctgacgaatattttttttttttttttttttctgtctcttatacacatctcacgtg

SEQ ID NO: 497 - DNA, 192 bp, Artificial sequence
  molecule of the complex
  misc_feature (119)..(119): s quence A permettant l'insertion d'une s quence compl mentaire d'un acide nucl ique d'int r t
agatgtgtataagagacagcacgtgttttttttttttttttttttcacgtgctgtctcttatacacatcttttctcgatcattattattttttggcgatcgcttttttttttttttttnttttttttttttttttgcgatcgcctttttttttttttttttttttagatgtgtataagagacaggacgaata

SEQ ID NO: 498 - DNA, 192 bp, Artificial sequence
  molecule of the complex
  misc_feature (119)..(119): s quence A permettant l'insertion d'une s quence compl mentaire d'un acide nucl ique d'int r t
ctgtctcttatacacatctcacgtgttttttttttttttttttttcacgtgagatgtgtataagagacagtttctcgatcattattattttttggcgatcgcttttttttttttttttnttttttttttttttttgcgatcgcctttttttttttttttttttttctgtctcttatacacatctgacgaata

SEQ ID NO: 499 - DNA, 186 bp, Artificial sequence
  molecule of the complex
  misc_feature (116)..(116): s quence A permettant l'insertion d'une s quence compl mentaire d'un acide nucl ique d'int r t
agatgtgtataagagacagcacgtgttttttttttttttttttttcacgtgctgtctcttatacacatcttttctcgatcattattattttttggtcgcttttttttttttttttnttttttttttttttttgcgacctttttttttttttttttttttagatgtgtataagagacaggacgaata

SEQ ID NO: 500 - DNA, 186 bp, Artificial sequence
  molecule of the complex
  misc_feature (116)..(116): s quence A permettant l'insertion d'une s quence compl mentaire d'un acide nucl ique d'int r t
ctgtctcttatacacatctcacgtgttttttttttttttttttttcacgtgagatgtgtataagagacagtttctcgatcattattattttttggtcgcttttttttttttttttnttttttttttttttttgcgacctttttttttttttttttttttctgtctcttatacacatctgacgaata

SEQ ID NO: 501 - DNA, 198 bp, Artificial sequence
  molecule of the complex
  misc_feature (122)..(122): s quence A permettant l'insertion d'une s quence compl mentaire d'un acide nucl ique d'int r t
agatgtgtataagagacagcacgtgttttttttttttttttttttcacgtgctgtctcttatacacatcttttctcgatcattattattttttgcggcgatcggcttttttttttttttttnttttttttttttttttgccgatcgccgctttttttttttttttttttttagatgtgtataagagacaggacgaata

SEQ ID NO: 502 - DNA, 198 bp, Artificial sequence
  molecule of the complex
  misc_feature (122)..(122): s quence A permettant l'insertion d'une s quence compl mentaire d'un acide nucl ique d'int r t
ctgtctcttatacacatctcacgtgttttttttttttttttttttcacgtgagatgtgtataagagacagtttctcgatcattattattttttgcggcgatcggcttttttttttttttttnttttttttttttttttgccgatcgccgctttttttttttttttttttttctgtctcttatacacatctgacgaata

SEQ ID NO: 503 - DNA, 95 bp, Artificial sequence; identical to SEQ ID NO: 8
  molecule of the complex
  misc_feature (95)..(95): replacement sequence

SEQ ID NO: 504 - DNA, 95 bp, Artificial sequence
  molecule of the complex
  misc_feature (95)..(95): replacement sequence
ctgtctcttatacacatctcagctgcagacaaagcttacagagatgtgtataagagacagttttttttttttttttttttttcatatgccaagtn

SEQ ID NO: 505 - DNA, 89 bp, Artificial sequence
  molecule of the complex
  misc_feature (83)..(83): replacement sequence
agatgtgtataagagacagcagctgcagacaaagcttacagctgtctcttatacacatctttttttttttttttttttttttnccaagt

SEQ ID NO: 506 - DNA, 89 bp, Artificial sequence
  molecule of the complex
  misc_feature (83)..(83): replacement sequence
ctgtctcttatacacatctcagctgcagacaaagcttacagagatgtgtataagagacagttttttttttttttttttttttnccaagt

SEQ ID NO: 507 - DNA, 99 bp, Artificial sequence
  molecule of the complex
  misc_feature (1)..(1): replacement sequence
ntacaagtccggataataattttttttttttttttttttttagatgtgtataagagacagctgggcacgcgtataagcagctgtctcttatacacatct

SEQ ID NO: 508 - DNA, 99 bp, Artificial sequence
  molecule of the complex
  misc_feature (1)..(1): replacement sequence
ntacaagtccggataataattttttttttttttttttttttctgtctcttatacacatctctgggcacgcgtataagcagagatgtgtataagagacag

SEQ ID NO: 509 - DNA, 93 bp, Artificial sequence
  molecule of the complex
  misc_feature (7)..(7): replacement sequence
tacaagntaataattttttttttttttttttttttagatgtgtataagagacagctgggcacgcgtataagcagctgtctcttatacacatct

SEQ ID NO: 510 - DNA, 93 bp, Artificial sequence
  molecule of the complex
  misc_feature (7)..(7): replacement sequence
tacaagntaataattttttttttttttttttttttctgtctcttatacacatctctgggcacgcgtataagcagagatgtgtataagagacag

SEQ ID NO: 511 - DNA, 93 bp, Artificial sequence
  molecule of the complex
  misc_feature (1)..(1): replacement sequence
ntacaagtaataattttttttttttttttttttttagatgtgtataagagacagctgggcacgcgtataagcagctgtctcttatacacatct

SEQ ID NO: 512 - DNA, 93 bp, Artificial sequence
  molecule of the complex
  misc_feature (1)..(1): replacement sequence
ntacaagtaataattttttttttttttttttttttctgtctcttatacacatctctgggcacgcgtataagcagagatgtgtataagagacag

SEQ ID NO: 513 - DNA, 64 bp, Artificial sequence; identical to SEQ ID NO: 10
  molecule of the complex
  misc_feature (1)..(1): replacement sequence

SEQ ID NO: 514 - DNA, 64 bp, Artificial sequence
  molecule of the complex
  misc_feature (1)..(1): replacement sequence
nacttggttaattaattttttttttttttttttttttctgtctcttatacacatctctactatc

SEQ ID NO: 515 - DNA, 64 bp, Artificial sequence
  molecule of the complex
  misc_feature (7)..(7): replacement sequence
acttggnttaattaattttttttttttttttttttttagatgtgtataagagacagctactatc

SEQ ID NO: 516 - DNA, 64 bp, Artificial sequence
  molecule of the complex
  misc_feature (7)..(7): replacement sequence
acttggnttaattaattttttttttttttttttttttctgtctcttatacacatctctactatc

SEQ ID NO: 517 - DNA, 70 bp, Artificial sequence
  molecule of the complex
  misc_feature (1)..(1): replacement sequence
nacttggcatatgttaattaattttttttttttttttttttttagatgtgtataagagacagctactatc

SEQ ID NO: 518 - DNA, 70 bp, Artificial sequence
  molecule of the complex
  misc_feature (1)..(1): replacement sequence
nacttggcatatgttaattaattttttttttttttttttttttctgtctcttatacacatctctactatc

SEQ ID NO: 519 - DNA, 63 bp, Artificial sequence
  molecule of the complex
  misc_feature (63)..(63): replacement sequence
tattcgtcctgtctcttatacacatctttttttttttttttttttattaattattacttgtan

SEQ ID NO: 520 - DNA, 63 bp, Artificial sequence
  molecule of the complex
  misc_feature (63)..(63): replacement sequence
tattcgtcagatgtgtataagagacagttttttttttttttttttattaattattacttgtan

SEQ ID NO: 521 - DNA, 63 bp, Artificial sequence
  molecule of the complex
  misc_feature (57)..(57): replacement sequence
tattcgtcctgtctcttatacacatctttttttttttttttttttattaattattancttgta

SEQ ID NO: 522 - DNA, 63 bp, Artificial sequence
  molecule of the complex
  misc_feature (57)..(57): replacement sequence
tattcgtcagatgtgtataagagacagttttttttttttttttttattaattattancttgta

SEQ ID NO: 523 - DNA, 69 bp, Artificial sequence
  molecule of the complex
  misc_feature (69)..(69): replacement sequence
tattcgtcctgtctcttatacacatctttttttttttttttttttattaattattatccggacttgtan

SEQ ID NO: 524 - DNA, 69 bp, Artificial sequence
  molecule of the complex
  misc_feature (69)..(69): replacement sequence
tattcgtcagatgtgtataagagacagttttttttttttttttttattaattattatccggacttgtan

SEQ ID NO: 525 - DNA, 167 bp, Artificial sequence
  molecule of the complex
  misc_feature (84)..(84): s quence A permettant l'insertion d'une s quence compl mentaire d'un acide nucl ique d'int r t
tgcagctgctgactcttatacacaagttttttttttttttttttttttttttttggcgatcgcttttttttttttttttttttnttttttttttttttttttttgcgatcgccttttttttttttttttgatacatgtttacttgtgtataagagtcagctgtaagc

SEQ ID NO: 526 - DNA, 167 bp, Artificial sequence
  molecule of the complex
  misc_feature (84)..(84): s quence A permettant l'insertion d'une s quence compl mentaire d'un acide nucl ique d'int r t
tgcagctgacttgtgtataagagtcagtttttttttttttttttttttttttttggcgatcgcttttttttttttttttttttnttttttttttttttttttttgcgatcgccttttttttttttttttgatacatgtttctgactcttatacacaagtctgtaagc

SEQ ID NO: 527 - DNA, 161 bp, Artificial sequence
  molecule of the complex
  misc_feature (81)..(81): s quence A permettant l'insertion d'une s quence compl mentaire d'un acide nucl ique d'int r t
tgcagctgctgactcttatacacaagttttttttttttttttttttttttttttggtcgcttttttttttttttttttttnttttttttttttttttttttgcgaccttttttttttttttttgatacatgtttacttgtgtataagagtcagctgtaagc

SEQ ID NO: 528 - DNA, 161 bp, Artificial sequence
  molecule of the complex
  misc_feature (81)..(81): s quence A permettant l'insertion d'une s quence compl mentaire d'un acide nucl ique d'int r t
tgcagctgacttgtgtataagagtcagtttttttttttttttttttttttttttggtcgcttttttttttttttttttttnttttttttttttttttttttgcgaccttttttttttttttttgatacatgtttctgactcttatacacaagtctgtaagc

SEQ ID NO: 529 - DNA, 173 bp, Artificial sequence
  molecule of the complex
  misc_feature (87)..(87): s quence A permettant l'insertion d'une s quence compl mentaire d'un acide nucl ique d'int r t
tgcagctgctgactcttatacacaagttttttttttttttttttttttttttttgcggcgatcggcttttttttttttttttttttnttttttttttttttttttttgccgatcgccgcttttttttttttttttgatacatgtttacttgtgtataagagtcagctgtaagc

SEQ ID NO: 530 - DNA, 173 bp, Artificial sequence
  molecule of the complex
  misc_feature (87)..(87): s quence A permettant l'insertion d'une s quence compl mentaire d'un acide nucl ique d'int r t
tgcagctgacttgtgtataagagtcagtttttttttttttttttttttttttttgcggcgatcggcttttttttttttttttttttnttttttttttttttttttttgccgatcgccgcttttttttttttttttgatacatgtttctgactcttatacacaagtctgtaagc

SEQ ID NO: 531 - DNA, 161 bp, Artificial sequence
  molecule of the complex
  misc_feature (81)..(81): s quence A permettant l'insertion d'une s quence compl mentaire d'un acide nucl ique d'int r t
gtgcccagctgactcttatacacaagttttctcgatcattttttttttttttttggtcgcttttttttttttttttttttnttttttttttttttttttttgcgacctttttttttttttttttttttttttttacttgtgtataagagtcagctgcttat

SEQ ID NO: 532 - DNA, 161 bp, Artificial sequence
  molecule of the complex
  misc_feature (81)..(81): s quence A permettant l'insertion d'une s quence compl mentaire d'un acide nucl ique d'int r t
gtgcccagacttgtgtataagagtcagtttctcgatcattttttttttttttttggtcgcttttttttttttttttttttnttttttttttttttttttttgcgacctttttttttttttttttttttttttttctgactcttatacacaagtctgcttat

SEQ ID NO: 533 - DNA, 189 bp, Artificial sequence
  molecule of the complex
  misc_feature (117)..(117): s quence A permettant l'insertion d'une s quence compl mentaire d'un acide nucl ique d'int r t
atcatcctgactcttatacacaagttttttttttttttttttgatagtagctgactcttatacacaagtttttttttttttttttttttttggcgatcgcttttttttttttttttnttttttttttttttttgcgatcgcctttttttttttttgatacatttacttgtgtataagagtcaggatgat

SEQ ID NO: 534 - DNA, 189 bp, Artificial sequence
  molecule of the complex
  misc_feature (117)..(117): s quence A permettant l'insertion d'une s quence compl mentaire d'un acide nucl ique d'int r t
atcatcacttgtgtataagagtcagtttttttttttttttttgatagtagacttgtgtataagagtcagttttttttttttttttttttttggcgatcgcttttttttttttttttnttttttttttttttttgcgatcgcctttttttttttttgatacatttctgactcttatacacaagtgatgat

SEQ ID NO: 535 - DNA, 183 bp, Artificial sequence
  molecule of the complex
  misc_feature (114)..(114): s quence A permettant l'insertion d'une s quence compl mentaire d'un acide nucl ique d'int r t
atcatcctgactcttatacacaagttttttttttttttttttgatagtagctgactcttatacacaagtttttttttttttttttttttttggtcgcttttttttttttttttnttttttttttttttttgcgacctttttttttttttgatacatttacttgtgtataagagtcaggatgat

SEQ ID NO: 536 - DNA, 183 bp, Artificial sequence
  molecule of the complex
  misc_feature (114)..(114): s quence A permettant l'insertion d'une s quence compl mentaire d'un acide nucl ique d'int r t
atcatcacttgtgtataagagtcagtttttttttttttttttgatagtagacttgtgtataagagtcagttttttttttttttttttttttggtcgcttttttttttttttttnttttttttttttttttgcgacctttttttttttttgatacatttctgactcttatacacaagtgatgat

SEQ ID NO: 537 - DNA, 195 bp, Artificial sequence
  molecule of the complex
  misc_feature (120)..(120): s quence A permettant l'insertion d'une s quence compl mentaire d'un acide nucl ique d'int r t
atcatcctgactcttatacacaagttttttttttttttttttgatagtagctgactcttatacacaagtttttttttttttttttttttttgcggcgatcggcttttttttttttttttnttttttttttttttttgccgatcgccgctttttttttttttgatacatttacttgtgtataagagtcaggatgat

SEQ ID NO: 538 - DNA, 195 bp, Artificial sequence
  molecule of the complex
  misc_feature (120)..(120): s quence A permettant l'insertion d'une s quence compl mentaire d'un acide nucl ique d'int r t
atcatcacttgtgtataagagtcagtttttttttttttttttgatagtagacttgtgtataagagtcagttttttttttttttttttttttgcggcgatcggcttttttttttttttttnttttttttttttttttgccgatcgccgctttttttttttttgatacatttctgactcttatacacaagtgatgat

SEQ ID NO: 539 - DNA, 189 bp, Artificial sequence
  molecule of the complex
  misc_feature (75)..(75): s quence A permettant l'insertion d'une s quence compl mentaire d'un acide nucl ique d'int r t
gatagtagctgactcttatacacaagtttttttttttttttttttttttggcgatcgcttttttttttttttttnttttttttttttttttgcgatcgcctttttttttttttgatacatttacttgtgtataagagtcaggatgattttttttttttttttttatcatcctgactcttatacacaagt

SEQ ID NO: 540 - DNA, 189 bp, Artificial sequence
  molecule of the complex
  misc_feature (75)..(75): s quence A permettant l'insertion d'une s quence compl mentaire d'un acide nucl ique d'int r t
gatagtagacttgtgtataagagtcagttttttttttttttttttttttggcgatcgcttttttttttttttttnttttttttttttttttgcgatcgcctttttttttttttgatacatttctgactcttatacacaagtgatgattttttttttttttttttatcatcacttgtgtataagagtcag

SEQ ID NO: 541 - DNA, 183 bp, Artificial sequence
  molecule of the complex
  misc_feature (72)..(72): s quence A permettant l'insertion d'une s quence compl mentaire d'un acide nucl ique d'int r t
gatagtagctgactcttatacacaagtttttttttttttttttttttttggtcgcttttttttttttttttnttttttttttttttttgcgacctttttttttttttgatacatttacttgtgtataagagtcaggatgattttttttttttttttttatcatcctgactcttatacacaagt

SEQ ID NO: 542 - DNA, 183 bp, Artificial sequence
  molecule of the complex
  misc_feature (72)..(72): s quence A permettant l'insertion d'une s quence compl mentaire d'un acide nucl ique d'int r t
gatagtagacttgtgtataagagtcagttttttttttttttttttttttggtcgcttttttttttttttttnttttttttttttttttgcgacctttttttttttttgatacatttctgactcttatacacaagtgatgattttttttttttttttttatcatcacttgtgtataagagtcag

SEQ ID NO: 543 - DNA, 195 bp, Artificial sequence
  molecule of the complex
  misc_feature (78)..(78): s quence A permettant l'insertion d'une s quence compl mentaire d'un acide nucl ique d'int r t
gatagtagctgactcttatacacaagtttttttttttttttttttttttgcggcgatcggcttttttttttttttttnttttttttttttttttgccgatcgccgctttttttttttttgatacatttacttgtgtataagagtcaggatgattttttttttttttttttatcatcctgactcttatacacaagt

SEQ ID NO: 544 - DNA, 195 bp, Artificial sequence
  molecule of the complex
  misc_feature (78)..(78): s quence A permettant l'insertion d'une s quence compl mentaire d'un acide nucl ique d'int r t
gatagtagacttgtgtataagagtcagttttttttttttttttttttttgcggcgatcggcttttttttttttttttnttttttttttttttttgccgatcgccgctttttttttttttgatacatttctgactcttatacacaagtgatgattttttttttttttttttatcatcacttgtgtataagagtcag

SEQ ID NO: 545 - DNA, 192 bp, Artificial sequence
  molecule of the complex
  misc_feature (74)..(74): s quence A permettant l'insertion d'une s quence compl mentaire d'un acide nucl ique d'int r t
cacgtgctgactcttatacacaagttttctcgatcattattattttttggcgatcgcttttttttttttttttnttttttttttttttttgcgatcgcctttttttttttttttttttttacttgtgtataagagtcaggacgaatattttttttttttttttttttacttgtgtataagagtcagcacgtg

SEQ ID NO: 546 - DNA, 192 bp, Artificial sequence
  molecule of the complex
  misc_feature (74)..(74): s quence A permettant l'insertion d'une s quence compl mentaire d'un acide nucl ique d'int r t
cacgtgacttgtgtataagagtcagtttctcgatcattattattttttggcgatcgcttttttttttttttttnttttttttttttttttgcgatcgcctttttttttttttttttttttctgactcttatacacaagtgacgaatattttttttttttttttttttctgactcttatacacaagtcacgtg

SEQ ID NO: 547 - DNA, 186 bp, Artificial sequence
  molecule of the complex
  misc_feature (71)..(71): s quence A permettant l'insertion d'une s quence compl mentaire d'un acide nucl ique d'int r t
cacgtgctgactcttatacacaagttttctcgatcattattattttttggtcgcttttttttttttttttnttttttttttttttttgcgacctttttttttttttttttttttacttgtgtataagagtcaggacgaatattttttttttttttttttttacttgtgtataagagtcagcacgtg

SEQ ID NO: 548 - DNA, 186 bp, Artificial sequence
  molecule of the complex
  misc_feature (71)..(71): s quence A permettant l'insertion d'une s quence compl mentaire d'un acide nucl ique d'int r t
cacgtgacttgtgtataagagtcagtttctcgatcattattattttttggtcgcttttttttttttttttnttttttttttttttttgcgacctttttttttttttttttttttctgactcttatacacaagtgacgaatattttttttttttttttttttctgactcttatacacaagtcacgtg

SEQ ID NO: 549 - DNA, 198 bp, Artificial sequence
  molecule of the complex
  misc_feature (77)..(77): s quence A permettant l'insertion d'une s quence compl mentaire d'un acide nucl ique d'int r t
cacgtgctgactcttatacacaagttttctcgatcattattattttttgcggcgatcggcttttttttttttttttnttttttttttttttttgccgatcgccgctttttttttttttttttttttacttgtgtataagagtcaggacgaatattttttttttttttttttttacttgtgtataagagtcagcacgtg

SEQ ID NO: 550 - DNA, 198 bp, Artificial sequence
  molecule of the complex
  misc_feature (77)..(77): s quence A permettant l'insertion d'une s quence compl mentaire d'un acide nucl ique d'int r t
cacgtgacttgtgtataagagtcagtttctcgatcattattattttttgcggcgatcggcttttttttttttttttnttttttttttttttttgccgatcgccgctttttttttttttttttttttctgactcttatacacaagtgacgaatattttttttttttttttttttctgactcttatacacaagtcacgtg

SEQ ID NO: 551 - DNA, 192 bp, Artificial sequence
  molecule of the complex
  misc_feature (119)..(119): s quence A permettant l'insertion d'une s quence compl mentaire d'un acide nucl ique d'int r t
acttgtgtataagagtcagcacgtgttttttttttttttttttttcacgtgctgactcttatacacaagttttctcgatcattattattttttggcgatcgcttttttttttttttttnttttttttttttttttgcgatcgcctttttttttttttttttttttacttgtgtataagagtcaggacgaata

SEQ ID NO: 552 - DNA, 192 bp, Artificial sequence
  molecule of the complex
  misc_feature (119)..(119): s quence A permettant l'insertion d'une s quence compl mentaire d'un acide nucl ique d'int r t
ctgactcttatacacaagtcacgtgttttttttttttttttttttcacgtgacttgtgtataagagtcagtttctcgatcattattattttttggcgatcgcttttttttttttttttnttttttttttttttttgcgatcgcctttttttttttttttttttttctgactcttatacacaagtgacgaata

SEQ ID NO: 553 - DNA, 186 bp, Artificial sequence
  molecule of the complex
  misc_feature (116)..(116): s quence A permettant l'insertion d'une s quence compl mentaire d'un acide nucl ique d'int r t
acttgtgtataagagtcagcacgtgttttttttttttttttttttcacgtgctgactcttatacacaagttttctcgatcattattattttttggtcgcttttttttttttttttnttttttttttttttttgcgacctttttttttttttttttttttacttgtgtataagagtcaggacgaata

SEQ ID NO: 554 - DNA, 186 bp, Artificial sequence
  molecule of the complex
  misc_feature (116)..(116): s quence A permettant l'insertion d'une s quence compl mentaire d'un acide nucl ique d'int r t
ctgactcttatacacaagtcacgtgttttttttttttttttttttcacgtgacttgtgtataagagtcagtttctcgatcattattattttttggtcgcttttttttttttttttnttttttttttttttttgcgacctttttttttttttttttttttctgactcttatacacaagtgacgaata

SEQ ID NO: 555 - DNA, 198 bp, Artificial sequence
  molecule of the complex
  misc_feature (122)..(122): s quence A permettant l'insertion d'une s quence compl mentaire d'un acide nucl ique d'int r t
acttgtgtataagagtcagcacgtgttttttttttttttttttttcacgtgctgactcttatacacaagttttctcgatcattattattttttgcggcgatcggcttttttttttttttttnttttttttttttttttgccgatcgccgctttttttttttttttttttttacttgtgtataagagtcaggacgaata

SEQ ID NO: 556 - DNA, 198 bp, Artificial sequence
  molecule of the complex
  misc_feature (122)..(122): s quence A permettant l'insertion d'une s quence compl mentaire d'un acide nucl ique d'int r t
ctgactcttatacacaagtcacgtgttttttttttttttttttttcacgtgacttgtgtataagagtcagtttctcgatcattattattttttgcggcgatcggcttttttttttttttttnttttttttttttttttgccgatcgccgctttttttttttttttttttttctgactcttatacacaagtgacgaata

SEQ ID NO: 557 - DNA, 95 bp, Artificial sequence
  molecule of the complex
  misc_feature (95)..(95): s quence A permettant l'insertion d'une s quence compl mentaire d'un acide nucl ique d'int r t
acttgtgtataagagtcagcagctgcagacaaagcttacagctgactcttatacacaagtttttttttttttttttttttttcatatgccaagtn

SEQ ID NO: 558 - DNA, 95 bp, Artificial sequence
  molecule of the complex
  misc_feature (95)..(95): s quence A permettant l'insertion d'une s quence compl mentaire d'un acide nucl ique d'int r t
ctgactcttatacacaagtcagctgcagacaaagcttacagacttgtgtataagagtcagttttttttttttttttttttttcatatgccaagtn

SEQ ID NO: 559 - DNA, 89 bp, Artificial sequence
  molecule of the complex
  misc_feature (83)..(83): s quence A permettant l'insertion d'une s quence compl mentaire d'un acide nucl ique d'int r t
acttgtgtataagagtcagcagctgcagacaaagcttacagctgactcttatacacaagtttttttttttttttttttttttnccaagt

SEQ ID NO: 560 - DNA, 89 bp, Artificial sequence
  molecule of the complex
  misc_feature (83)..(83): s quence A permettant l'insertion d'une s quence compl mentaire d'un acide nucl ique d'int r t
ctgactcttatacacaagtcagctgcagacaaagcttacagacttgtgtataagagtcagttttttttttttttttttttttnccaagt

SEQ ID NO: 561 - DNA, 99 bp, Artificial sequence
  molecule of the complex
  misc_feature (1)..(1): replacement sequence
ntacaagtccggataataattttttttttttttttttttttacttgtgtataagagtcagctgggcacgcgtataagcagctgactcttatacacaagt

SEQ ID NO: 562 - DNA, 99 bp, Artificial sequence
  molecule of the complex
  misc_feature (1)..(1): replacement sequence
ntacaagtccggataataattttttttttttttttttttttctgactcttatacacaagtctgggcacgcgtataagcagacttgtgtataagagtcag

SEQ ID NO: 563 - DNA, 93 bp, Artificial sequence
  molecule of the complex
  misc_feature (7)..(7): replacement sequence
tacaagntaataattttttttttttttttttttttacttgtgtataagagtcagctgggcacgcgtataagcagctgactcttatacacaagt

SEQ ID NO: 564 - DNA, 93 bp, Artificial sequence
  molecule of the complex
  misc_feature (7)..(7): replacement sequence
tacaagntaataattttttttttttttttttttttctgactcttatacacaagtctgggcacgcgtataagcagacttgtgtataagagtcag

SEQ ID NO: 565 - DNA, 93 bp, Artificial sequence
  molecule of the complex
  misc_feature (1)..(1): replacement sequence
ntacaagtaataattttttttttttttttttttttacttgtgtataagagtcagctgggcacgcgtataagcagctgactcttatacacaagt

SEQ ID NO: 566 - DNA, 93 bp, Artificial sequence
  molecule of the complex
  misc_feature (1)..(1): replacement sequence
ntacaagtaataattttttttttttttttttttttctgactcttatacacaagtctgggcacgcgtataagcagacttgtgtataagagtcag

SEQ ID NO: 567 - DNA, 64 bp, Artificial sequence
  molecule of the complex
  misc_feature (1)..(1): replacement sequence
nacttggttaattaattttttttttttttttttttttacttgtgtataagagtcagctactatc

SEQ ID NO: 568 - DNA, 64 bp, Artificial sequence
  molecule of the complex
  misc_feature (1)..(1): replacement sequence
nacttggttaattaattttttttttttttttttttttctgactcttatacacaagtctactatc

SEQ ID NO: 569 - DNA, 64 bp, Artificial sequence
  molecule of the complex
  misc_feature (7)..(7): replacement sequence
acttggnttaattaattttttttttttttttttttttacttgtgtataagagtcagctactatc

SEQ ID NO: 570 - DNA, 64 bp, Artificial sequence
  molecule of the complex
  misc_feature (7)..(7): replacement sequence
acttggnttaattaattttttttttttttttttttttctgactcttatacacaagtctactatc

SEQ ID NO: 571 - DNA, 70 bp, Artificial sequence
  molecule of the complex
  misc_feature (1)..(1): replacement sequence
nacttggcatatgttaattaattttttttttttttttttttttacttgtgtataagagtcagctactatc

SEQ ID NO: 572 - DNA, 70 bp, Artificial sequence
  molecule of the complex
  misc_feature (1)..(1): replacement sequence
nacttggcatatgttaattaattttttttttttttttttttttctgactcttatacacaagtctactatc

SEQ ID NO: 573 - DNA, 63 bp, Artificial sequence
  molecule of the complex
  misc_feature (63)..(63): replacement sequence
tattcgtcctgactcttatacacaagtttttttttttttttttttattaattattacttgtan

SEQ ID NO: 574 - DNA, 63 bp, Artificial sequence
  molecule of the complex
  misc_feature (63)..(63): replacement sequence
tattcgtcacttgtgtataagagtcagttttttttttttttttttattaattattacttgtan

SEQ ID NO: 575 - DNA, 63 bp, Artificial sequence
  molecule of the complex
  misc_feature (57)..(57): replacement sequence
tattcgtcctgactcttatacacaagtttttttttttttttttttattaattattancttgta

SEQ ID NO: 576 - DNA, 63 bp, Artificial sequence
  molecule of the complex
  misc_feature (57)..(57): replacement sequence
tattcgtcacttgtgtataagagtcagttttttttttttttttttattaattattancttgta

SEQ ID NO: 577 - DNA, 69 bp, Artificial sequence
  molecule of the complex
  misc_feature (69)..(69): replacement sequence
tattcgtcctgactcttatacacaagtttttttttttttttttttattaattattatccggacttgtan

SEQ ID NO: 578 - DNA, 69 bp, Artificial sequence
  molecule of the complex
  misc_feature (69)..(69): replacement sequence
tattcgtcacttgtgtataagagtcagttttttttttttttttttattaattattatccggacttgtan

SEQ ID NO: 579 - DNA, 167 bp, Artificial sequence
  molecule of the complex
  misc_feature (84)..(84): replacement sequence
tgcagctgctgtctcttgatcagatcttttttttttttttttttttttttttttggcgatcgcttttttttttttttttttttnttttttttttttttttttttgcgatcgccttttttttttttttttgatacatgtttagatctgatcaagagacagctgtaagc

SEQ ID NO: 580 - DNA, 167 bp, Artificial sequence
  molecule of the complex
  misc_feature (84)..(84): replacement sequence
tgcagctgagatctgatcaagagacagtttttttttttttttttttttttttttggcgatcgcttttttttttttttttttttnttttttttttttttttttttgcgatcgccttttttttttttttttgatacatgtttctgtctcttgatcagatctctgtaagc

SEQ ID NO: 581 - DNA, 161 bp, Artificial sequence
  molecule of the complex
  misc_feature (81)..(81): replacement sequence
tgcagctgctgtctcttgatcagatcttttttttttttttttttttttttttttggtcgcttttttttttttttttttttnttttttttttttttttttttgcgaccttttttttttttttttgatacatgtttagatctgatcaagagacagctgtaagc

SEQ ID NO: 582 - DNA, 161 bp, Artificial sequence
  molecule of the complex
  misc_feature (81)..(81): replacement sequence
tgcagctgagatctgatcaagagacagtttttttttttttttttttttttttttggtcgcttttttttttttttttttttnttttttttttttttttttttgcgaccttttttttttttttttgatacatgtttctgtctcttgatcagatctctgtaagc

SEQ ID NO: 583 - DNA, 173 bp, Artificial sequence
  molecule of the complex
  misc_feature (87)..(87): s quence A permettant l'insertion d'une s quence compl mentaire d'un acide nucl ique d'int r t
tgcagctgctgtctcttgatcagatcttttttttttttttttttttttttttttgcggcgatcggcttttttttttttttttttttnttttttttttttttttttttgccgatcgccgcttttttttttttttttgatacatgtttagatctgatcaagagacagctgtaagc

SEQ ID NO: 584 - DNA, 173 bp, Artificial sequence
  molecule of the complex
  misc_feature (87)..(87): s quence A permettant l'insertion d'une s quence compl mentaire d'un acide nucl ique d'int r t
tgcagctgagatctgatcaagagacagtttttttttttttttttttttttttttgcggcgatcggcttttttttttttttttttttnttttttttttttttttttttgccgatcgccgcttttttttttttttttgatacatgtttctgtctcttgatcagatctctgtaagc

SEQ ID NO: 585 - DNA, 161 bp, Artificial sequence
  molecule of the complex
  misc_feature (81)..(81): s quence A permettant l'insertion d'une s quence compl mentaire d'un acide nucl ique d'int r t
gtgcccagctgtctcttgatcagatcttttctcgatcattttttttttttttttggtcgcttttttttttttttttttttnttttttttttttttttttttgcgacctttttttttttttttttttttttttttagatctgatcaagagacagctgcttat

SEQ ID NO: 586 - DNA, 161 bp, Artificial sequence
  molecule of the complex
  misc_feature (81)..(81): s quence A permettant l'insertion d'une s quence compl mentaire d'un acide nucl ique d'int r t
gtgcccagagatctgatcaagagacagtttctcgatcattttttttttttttttggtcgcttttttttttttttttttttnttttttttttttttttttttgcgacctttttttttttttttttttttttttttctgtctcttgatcagatctctgcttat

SEQ ID NO: 587 - DNA, 167 bp, Artificial sequence
  molecule of the complex
  misc_feature (84)..(84): s quence A permettant l'insertion d'une s quence compl mentaire d'un acide nucl ique d'int r t
gtgcccagctgtctcttgatcagatcttttctcgatcattttttttttttttttggcgatcgcttttttttttttttttttttnttttttttttttttttttttgcgatcgcctttttttttttttttttttttttttttagatctgatcaagagacagctgcttat

SEQ ID NO: 588 - DNA, 167 bp, Artificial sequence
  molecule of the complex
  misc_feature (84)..(84): s quence A permettant l'insertion d'une s quence compl mentaire d'un acide nucl ique d'int r t
gtgcccagagatctgatcaagagacagtttctcgatcattttttttttttttttggcgatcgcttttttttttttttttttttnttttttttttttttttttttgcgatcgcctttttttttttttttttttttttttttctgtctcttgatcagatctctgcttat

SEQ ID NO: 589 - DNA, 173 bp, Artificial sequence
  molecule of the complex
  misc_feature (87)..(87): s quence A permettant l'insertion d'une s quence compl mentaire d'un acide nucl ique d'int r t
gtgcccagctgtctcttgatcagatcttttctcgatcattttttttttttttttgcggcgatcggcttttttttttttttttttttnttttttttttttttttttttgccgatcgccgctttttttttttttttttttttttttttagatctgatcaagagacagctgcttat

SEQ ID NO: 590 - DNA, 173 bp, Artificial sequence
  molecule of the complex
  misc_feature (87)..(87): s quence A permettant l'insertion d'une s quence compl mentaire d'un acide nucl ique d'int r t
gtgcccagagatctgatcaagagacagtttctcgatcattttttttttttttttgcggcgatcggcttttttttttttttttttttnttttttttttttttttttttgccgatcgccgctttttttttttttttttttttttttttctgtctcttgatcagatctctgcttat

SEQ ID NO: 591 - DNA, 189 bp, Artificial sequence
  molecule of the complex
  misc_feature (117)..(117): s quence A permettant l'insertion d'une s quence compl mentaire d'un acide nucl ique d'int r t
atcatcctgtctcttgatcagatcttttttttttttttttttgatagtagctgtctcttgatcagatctttttttttttttttttttttttggcgatcgcttttttttttttttttnttttttttttttttttgcgatcgcctttttttttttttgatacatttagatctgatcaagagacaggatgat

SEQ ID NO: 592 - DNA, 189 bp, Artificial sequence
  molecule of the complex
  misc_feature (117)..(117): s quence A permettant l'insertion d'une s quence compl mentaire d'un acide nucl ique d'int r t
atcatcagatctgatcaagagacagtttttttttttttttttgatagtagagatctgatcaagagacagttttttttttttttttttttttggcgatcgcttttttttttttttttnttttttttttttttttgcgatcgcctttttttttttttgatacatttctgtctcttgatcagatctgatgat

SEQ ID NO: 593 - DNA, 183 bp, Artificial sequence
  molecule of the complex
  misc_feature (114)..(114): s quence A permettant l'insertion d'une s quence compl mentaire d'un acide nucl ique d'int r t
atcatcctgtctcttgatcagatcttttttttttttttttttgatagtagctgtctcttgatcagatctttttttttttttttttttttttggtcgcttttttttttttttttnttttttttttttttttgcgacctttttttttttttgatacatttagatctgatcaagagacaggatgat

SEQ ID NO: 594 - DNA, 183 bp, Artificial sequence
  molecule of the complex
  misc_feature (114)..(114): s quence A permettant l'insertion d'une s quence compl mentaire d'un acide nucl ique d'int r t
atcatcagatctgatcaagagacagtttttttttttttttttgatagtagagatctgatcaagagacagttttttttttttttttttttttggtcgcttttttttttttttttnttttttttttttttttgcgacctttttttttttttgatacatttctgtctcttgatcagatctgatgat

SEQ ID NO: 595 - DNA, 195 bp, Artificial sequence
  molecule of the complex
  misc_feature (120)..(120): s quence A permettant l'insertion d'une s quence compl mentaire d'un acide nucl ique d'int r t
atcatcctgtctcttgatcagatcttttttttttttttttttgatagtagctgtctcttgatcagatctttttttttttttttttttttttgcggcgatcggcttttttttttttttttnttttttttttttttttgccgatcgccgctttttttttttttgatacatttagatctgatcaagagacaggatgat

SEQ ID NO: 596 - DNA, 195 bp, Artificial sequence
  molecule of the complex
  misc_feature (120)..(120): s quence A permettant l'insertion d'une s quence compl mentaire d'un acide nucl ique d'int r t
atcatcagatctgatcaagagacagtttttttttttttttttgatagtagagatctgatcaagagacagttttttttttttttttttttttgcggcgatcggcttttttttttttttttnttttttttttttttttgccgatcgccgctttttttttttttgatacatttctgtctcttgatcagatctgatgat

SEQ ID NO: 597 - DNA, 189 bp, Artificial sequence
  molecule of the complex
  misc_feature (75)..(75): s quence A permettant l'insertion d'une s quence compl mentaire d'un acide nucl ique d'int r t
gatagtagctgtctcttgatcagatctttttttttttttttttttttttggcgatcgcttttttttttttttttnttttttttttttttttgcgatcgcctttttttttttttgatacatttagatctgatcaagagacaggatgattttttttttttttttttatcatcctgtctcttgatcagatct

SEQ ID NO: 598 - DNA, 189 bp, Artificial sequence
  molecule of the complex
  misc_feature (75)..(75): s quence A permettant l'insertion d'une s quence compl mentaire d'un acide nucl ique d'int r t
gatagtagagatctgatcaagagacagttttttttttttttttttttttggcgatcgcttttttttttttttttnttttttttttttttttgcgatcgcctttttttttttttgatacatttctgtctcttgatcagatctgatgattttttttttttttttttatcatcagatctgatcaagagacag

SEQ ID NO: 599 - DNA, 183 bp, Artificial sequence
  molecule of the complex
  misc_feature (72)..(72): s quence A permettant l'insertion d'une s quence compl mentaire d'un acide nucl ique d'int r t
gatagtagctgtctcttgatcagatctttttttttttttttttttttttggtcgcttttttttttttttttnttttttttttttttttgcgacctttttttttttttgatacatttagatctgatcaagagacaggatgattttttttttttttttttatcatcctgtctcttgatcagatct

SEQ ID NO: 600 - DNA, 183 bp, Artificial sequence
  molecule of the complex
  misc_feature (72)..(72): s quence A permettant l'insertion d'une s quence compl mentaire d'un acide nucl ique d'int r t
gatagtagagatctgatcaagagacagttttttttttttttttttttttggtcgcttttttttttttttttnttttttttttttttttgcgacctttttttttttttgatacatttctgtctcttgatcagatctgatgattttttttttttttttttatcatcagatctgatcaagagacag

SEQ ID NO: 601 - DNA, 195 bp, Artificial sequence
  molecule of the complex
  misc_feature (78)..(78): s quence A permettant l'insertion d'une s quence compl mentaire d'un acide nucl ique d'int r t
gatagtagctgtctcttgatcagatctttttttttttttttttttttttgcggcgatcggcttttttttttttttttnttttttttttttttttgccgatcgccgctttttttttttttgatacatttagatctgatcaagagacaggatgattttttttttttttttttatcatcctgtctcttgatcagatct

SEQ ID NO: 602 - DNA, 195 bp, Artificial sequence
  molecule of the complex
  misc_feature (78)..(78): s quence A permettant l'insertion d'une s quence compl mentaire d'un acide nucl ique d'int r t
gatagtagagatctgatcaagagacagttttttttttttttttttttttgcggcgatcggcttttttttttttttttnttttttttttttttttgccgatcgccgctttttttttttttgatacatttctgtctcttgatcagatctgatgattttttttttttttttttatcatcagatctgatcaagagacag

SEQ ID NO: 603 - DNA, 192 bp, Artificial sequence
  molecule of the complex
  misc_feature (74)..(74): s quence A permettant l'insertion d'une s quence compl mentaire d'un acide nucl ique d'int r t
cacgtgctgtctcttgatcagatcttttctcgatcattattattttttggcgatcgcttttttttttttttttnttttttttttttttttgcgatcgcctttttttttttttttttttttagatctgatcaagagacaggacgaatattttttttttttttttttttagatctgatcaagagacagcacgtg

SEQ ID NO: 604 - DNA, 192 bp, Artificial sequence
  molecule of the complex
  misc_feature (74)..(74): s quence A permettant l'insertion d'une s quence compl mentaire d'un acide nucl ique d'int r t
cacgtgagatctgatcaagagacagtttctcgatcattattattttttggcgatcgcttttttttttttttttnttttttttttttttttgcgatcgcctttttttttttttttttttttctgtctcttgatcagatctgacgaatattttttttttttttttttttctgtctcttgatcagatctcacgtg

SEQ ID NO: 605 - DNA, 186 bp, Artificial sequence
  molecule of the complex
  misc_feature (71)..(71): s quence A permettant l'insertion d'une s quence compl mentaire d'un acide nucl ique d'int r t
cacgtgctgtctcttgatcagatcttttctcgatcattattattttttggtcgcttttttttttttttttnttttttttttttttttgcgacctttttttttttttttttttttagatctgatcaagagacaggacgaatattttttttttttttttttttagatctgatcaagagacagcacgtg

SEQ ID NO: 606 - DNA, 186 bp, Artificial sequence
  molecule of the complex
  misc_feature (71)..(71): s quence A permettant l'insertion d'une s quence compl mentaire d'un acide nucl ique d'int r t
cacgtgagatctgatcaagagacagtttctcgatcattattattttttggtcgcttttttttttttttttnttttttttttttttttgcgacctttttttttttttttttttttctgtctcttgatcagatctgacgaatattttttttttttttttttttctgtctcttgatcagatctcacgtg

SEQ ID NO: 607 - DNA, 198 bp, Artificial sequence
  molecule of the complex
  misc_feature (77)..(77): s quence A permettant l'insertion d'une s quence compl mentaire d'un acide nucl ique d'int r t
cacgtgctgtctcttgatcagatcttttctcgatcattattattttttgcggcgatcggcttttttttttttttttnttttttttttttttttgccgatcgccgctttttttttttttttttttttagatctgatcaagagacaggacgaatattttttttttttttttttttagatctgatcaagagacagcacgtg

SEQ ID NO: 608 - DNA, 198 bp, Artificial sequence
  molecule of the complex
  misc_feature (77)..(77): s quence A permettant l'insertion d'une s quence compl mentaire d'un acide nucl ique d'int r t
cacgtgagatctgatcaagagacagtttctcgatcattattattttttgcggcgatcggcttttttttttttttttnttttttttttttttttgccgatcgccgctttttttttttttttttttttctgtctcttgatcagatctgacgaatattttttttttttttttttttctgtctcttgatcagatctcacgtg

SEQ ID NO: 609 - DNA, 192 bp, Artificial sequence
  molecule of the complex
  misc_feature (119)..(119): s quence A permettant l'insertion d'une s quence compl mentaire d'un acide nucl ique d'int r t
agatctgatcaagagacagcacgtgttttttttttttttttttttcacgtgctgtctcttgatcagatcttttctcgatcattattattttttggcgatcgcttttttttttttttttnttttttttttttttttgcgatcgcctttttttttttttttttttttagatctgatcaagagacaggacgaata

SEQ ID NO: 610 - DNA, 192 bp, Artificial sequence
  molecule of the complex
  misc_feature (119)..(119): s quence A permettant l'insertion d'une s quence compl mentaire d'un acide nucl ique d'int r t
ctgtctcttgatcagatctcacgtgttttttttttttttttttttcacgtgagatctgatcaagagacagtttctcgatcattattattttttggcgatcgcttttttttttttttttnttttttttttttttttgcgatcgcctttttttttttttttttttttctgtctcttgatcagatctgacgaata

SEQ ID NO: 611 - DNA, 186 bp, Artificial sequence
  molecule of the complex
  misc_feature (116)..(116): s quence A permettant l'insertion d'une s quence compl mentaire d'un acide nucl ique d'int r t
agatctgatcaagagacagcacgtgttttttttttttttttttttcacgtgctgtctcttgatcagatcttttctcgatcattattattttttggtcgcttttttttttttttttnttttttttttttttttgcgacctttttttttttttttttttttagatctgatcaagagacaggacgaata

SEQ ID NO: 612 - DNA, 186 bp, Artificial sequence
  molecule of the complex
  misc_feature (116)..(116): s quence A permettant l'insertion d'une s quence compl mentaire d'un acide nucl ique d'int r t
ctgtctcttgatcagatctcacgtgttttttttttttttttttttcacgtgagatctgatcaagagacagtttctcgatcattattattttttggtcgcttttttttttttttttnttttttttttttttttgcgacctttttttttttttttttttttctgtctcttgatcagatctgacgaata

SEQ ID NO: 613 - DNA, 198 bp, Artificial sequence
  molecule of the complex
  misc_feature (122)..(122): s quence A permettant l'insertion d'une s quence compl mentaire d'un acide nucl ique d'int r t
agatctgatcaagagacagcacgtgttttttttttttttttttttcacgtgctgtctcttgatcagatcttttctcgatcattattattttttgcggcgatcggcttttttttttttttttnttttttttttttttttgccgatcgccgctttttttttttttttttttttagatctgatcaagagacaggacgaata

SEQ ID NO: 614 - DNA, 198 bp, Artificial sequence
  molecule of the complex
  misc_feature (122)..(122): s quence A permettant l'insertion d'une s quence compl mentaire d'un acide nucl ique d'int r t
ctgtctcttgatcagatctcacgtgttttttttttttttttttttcacgtgagatctgatcaagagacagtttctcgatcattattattttttgcggcgatcggcttttttttttttttttnttttttttttttttttgccgatcgccgctttttttttttttttttttttctgtctcttgatcagatctgacgaata

SEQ ID NO: 615 - DNA, 95 bp, Artificial sequence
  molecule of the complex
  misc_feature (95)..(95): s quence A permettant l'insertion d'une s quence compl mentaire d'un acide nucl ique d'int r t
agatctgatcaagagacagcagctgcagacaaagcttacagctgtctcttgatcagatctttttttttttttttttttttttcatatgccaagtn

SEQ ID NO: 616 - DNA, 95 bp, Artificial sequence
  molecule of the complex
  misc_feature (95)..(95): s quence A permettant l'insertion d'une s quence compl mentaire d'un acide nucl ique d'int r t
ctgtctcttgatcagatctcagctgcagacaaagcttacagagatctgatcaagagacagttttttttttttttttttttttcatatgccaagtn

SEQ ID NO: 617 - DNA, 89 bp, Artificial sequence
  molecule of the complex
  misc_feature (83)..(83): s quence A permettant l'insertion d'une s quence compl mentaire d'un acide nucl ique d'int r t
agatctgatcaagagacagcagctgcagacaaagcttacagctgtctcttgatcagatctttttttttttttttttttttttnccaagt

SEQ ID NO: 618 - DNA, 89 bp, Artificial sequence
  molecule of the complex
  misc_feature (83)..(83): s quence A permettant l'insertion d'une s quence compl mentaire d'un acide nucl ique d'int r t
ctgtctcttgatcagatctcagctgcagacaaagcttacagagatctgatcaagagacagttttttttttttttttttttttnccaagt

SEQ ID NO: 619 - DNA, 99 bp, Artificial sequence
  molecule of the complex
  misc_feature (1)..(1): replacement sequence
ntacaagtccggataataattttttttttttttttttttttagatctgatcaagagacagctgggcacgcgtataagcagctgtctcttgatcagatct

SEQ ID NO: 620 - DNA, 99 bp, Artificial sequence
  molecule of the complex
  misc_feature (1)..(1): replacement sequence
ntacaagtccggataataattttttttttttttttttttttctgtctcttgatcagatctctgggcacgcgtataagcagagatctgatcaagagacag

SEQ ID NO: 621 - DNA, 93 bp, Artificial sequence
  molecule of the complex
  misc_feature (7)..(7): replacement sequence
tacaagntaataattttttttttttttttttttttagatctgatcaagagacagctgggcacgcgtataagcagctgtctcttgatcagatct

SEQ ID NO: 622 - DNA, 93 bp, Artificial sequence
  molecule of the complex
  misc_feature (7)..(7): replacement sequence
tacaagntaataattttttttttttttttttttttctgtctcttgatcagatctctgggcacgcgtataagcagagatctgatcaagagacag

SEQ ID NO: 623 - DNA, 93 bp, Artificial sequence
  molecule of the complex
  misc_feature (1)..(1): replacement sequence
ntacaagtaataattttttttttttttttttttttagatctgatcaagagacagctgggcacgcgtataagcagctgtctcttgatcagatct

SEQ ID NO: 624 - DNA, 93 bp, Artificial sequence
  molecule of the complex
  misc_feature (1)..(1): replacement sequence
ntacaagtaataattttttttttttttttttttttctgtctcttgatcagatctctgggcacgcgtataagcagagatctgatcaagagacag

SEQ ID NO: 625 - DNA, 64 bp, Artificial sequence
  molecule of the complex
  misc_feature (1)..(1): replacement sequence
nacttggttaattaattttttttttttttttttttttagatctgatcaagagacagctactatc

SEQ ID NO: 626 - DNA, 64 bp, Artificial sequence
  molecule of the complex
  misc_feature (1)..(1): replacement sequence
nacttggttaattaattttttttttttttttttttttctgtctcttgatcagatctctactatc

SEQ ID NO: 627 - DNA, 64 bp, Artificial sequence
  molecule of the complex
  misc_feature (7)..(7): replacement sequence
acttggnttaattaattttttttttttttttttttttagatctgatcaagagacagctactatc

SEQ ID NO: 628 - DNA, 64 bp, Artificial sequence
  molecule of the complex
  misc_feature (7)..(7): replacement sequence
acttggnttaattaattttttttttttttttttttttctgtctcttgatcagatctctactatc

SEQ ID NO: 629 - DNA, 70 bp, Artificial sequence
  molecule of the complex
  misc_feature (1)..(1): replacement sequence
nacttggcatatgttaattaattttttttttttttttttttttagatctgatcaagagacagctactatc

SEQ ID NO: 630 - DNA, 70 bp, Artificial sequence
  molecule of the complex
  misc_feature (1)..(1): replacement sequence
nacttggcatatgttaattaattttttttttttttttttttttctgtctcttgatcagatctctactatc

SEQ ID NO: 631 - DNA, 63 bp, Artificial sequence
  molecule of the complex
  misc_feature (63)..(63): replacement sequence
tattcgtcctgtctcttgatcagatctttttttttttttttttttattaattattacttgtan

SEQ ID NO: 632 - DNA, 63 bp, Artificial sequence
  molecule of the complex
  misc_feature (63)..(63): replacement sequence
tattcgtcagatctgatcaagagacagttttttttttttttttttattaattattacttgtan

SEQ ID NO: 633 - DNA, 63 bp, Artificial sequence
  molecule of the complex
  misc_feature (57)..(57): replacement sequence
tattcgtcctgtctcttgatcagatctttttttttttttttttttattaattattancttgta

SEQ ID NO: 634 - DNA, 63 bp, Artificial sequence
  molecule of the complex
  misc_feature (57)..(57): replacement sequence
tattcgtcagatctgatcaagagacagttttttttttttttttttattaattattancttgta

SEQ ID NO: 635 - DNA, 69 bp, Artificial sequence
  molecule of the complex
  misc_feature (69)..(69): replacement sequence
tattcgtcctgtctcttgatcagatctttttttttttttttttttattaattattatccggacttgtan

SEQ ID NO: 636 - DNA, 69 bp, Artificial sequence
  molecule of the complex
  misc_feature (69)..(69): replacement sequence
tattcgtcagatctgatcaagagacagttttttttttttttttttattaattattatccggacttgtan

SEQ ID NO: 637 - DNA, 63 bp, Artificial sequence; identical to SEQ ID NO: 633
  molecule of the complex
  misc_feature (57)..(57): replacement sequence

SEQ ID NO: 638 - DNA, 63 bp, Artificial sequence; identical to SEQ ID NO: 634
  molecule of the complex
  misc_feature (57)..(57): replacement sequence

SEQ ID NO: 639 - DNA, 69 bp, Artificial sequence; identical to SEQ ID NO: 635
  molecule of the complex
  misc_feature (69)..(69): replacement sequence

SEQ ID NO: 640 - DNA, 69 bp, Artificial sequence; identical to SEQ ID NO: 636
  molecule of the complex
  misc_feature (69)..(69): replacement sequence

SEQ ID NO: 641 - DNA, 136 bp, Artificial sequence
  molecule of the complex
  misc_feature (7)..(7): transposase binding site
  misc_feature (33)..(33): transposase binding site
  misc_feature (82)..(82): s quence A permettant l'insertion d'une s quence compl mentaire d'un acide nucl ique d'int r t
  misc_feature (130)..(130): transposase binding site
atcatcntttttttttttttttttgatagtagntttttttttttttttttttttttggcgatcgcttttttttttttttttnttttttttttttttttgcgatcgcctttttttttttttgatacatttngatgat

SEQ ID NO: 642 - DNA, 46 bp, Artificial sequence; identical to SEQ ID NO: 451
  molecule of the complex
  misc_feature (1)..(1): replacement sequence
  misc_feature (38)..(38): transposase binding site

SEQ ID NO: 643 - DNA, 131 bp, Artificial sequence; identical to SEQ ID NO: 436
  molecule of the complex
  misc_feature (9)..(9): transposase binding site
  misc_feature (66)..(66): s quence A permettant l'insertion d'une s quence compl mentaire d'un acide nucl ique d'int r t
  misc_feature (123)..(123): transposase binding site

SEQ ID NO: 644 - DNA, 59 bp, Artificial sequence; identical to SEQ ID NO: 437
  molecule of the complex
  misc_feature (1)..(1): transposase binding site
  misc_feature (24)..(24): transposase binding site
  misc_feature (59)..(59): replacement sequence

SEQ ID NO: 645 - DNA, 136 bp, Artificial sequence; identical to SEQ ID NO: 641
  molecule of the complex
  misc_feature (7)..(7): transposase binding site
  misc_feature (33)..(33): transposase binding site
  misc_feature (82)..(82): s quence A permettant l'insertion d'une s quence compl mentaire d'un acide nucl ique d'int r t
  misc_feature (130)..(130): transposase binding site

SEQ ID NO: 646 - DNA, 46 bp, Artificial sequence; identical to SEQ ID NO: 451
  molecule of the complex
  misc_feature (1)..(1): replacement sequence
  misc_feature (38)..(38): transposase binding site